European Patent Application EP 4 502 162 A1, published February 5, 2025. Title: Selective regulatory gene (SRG) system for gene-modified immune cell therapy. Applicant: 学校法人自治医科大学. The sequence listing filed with the application follows.

SEQUENCE LISTING (74 sequences)

SEQ ID NO: 1 - protein, 396 aa, synthetic construct
  REGION 1..396: note = TEG amino acid sequence
RAKRGKPIPNPLLGLDSTSGSGEGRGSLLTCGDVEENPGPDHLGASLWPQVGSLCLLLAGAAWAPPPNLPDPKFESKAALLAARGPEELLCFTERLEDLVCFWEEAASAGVGPGNYSFSYQLEDEPWKLCRLHQAPTARGAVRFWCSLPTADTSSFVPLELRVTAASGAPRYHRVIHINEVVLLDAPVGLVARLADESGHVVLRWLPPPETPMTSHIRYEVDVSAGNGAGSVQRVEILEGRTECVLSNLRGRTRYTFAVRARMAEPSFGGFWSAWSEPVSLLTPSDLDPVVISVGSMGLIISLLCVYFWLERTMPRIPTLKNLEDLVTEYHGNFSAWSGVSKGLAESLQPDYSERLCLVSEIPPKGGALGEGPGASPCNQHSPYWAPPCYTLKPET

SEQ ID NO: 2 - DNA, 1188 bp, synthetic construct
  misc_feature 1..1188: note = TEG nucleic acid sequence
  source 1..1188: mol_type = other DNA
agggccaagaggggcaagcccattcctaatcctctgctgggcctcgatagcacaagcggcagcggagaaggcagaggctctctgcttacatgcggcgacgtggaagagaaccccggacctgatcacctgggcgcttctctgtggcctcaagtgggatctctgtgtctgctgcttgctggcgctgcttgggctcctcctcctaatctgcccgatcctaagttcgagagcaaggccgctctgctggctgctagaggacctgaggaactgctgtgcttcaccgagagactcgaggacctcgtgtgcttctgggaagaagctgcttctgccggcgttggccctggcaattacagcttcagctaccagctggaagatgagccctggaagctgtgcagactgcatcaggcccctacagctagaggcgctgtgcggttttggtgtagcctgcctacagccgacaccagcagcttcgtgcctctggaactgagagtgacagccgcttctggcgcccctagataccacagagtgatccacatcaacgaggtggtgctgctggatgcccctgttggactggttgccagactggccgatgagtctggacatgtggtgctgagatggctgcctcctccagagacacctatgaccagccacatcagatacgaggtggacgtgtccgccggaaatggcgctggatctgtgcagagagtggaaatcctggaaggccggaccgagtgcgtgctgagcaatctgagaggcagaacccggtacaccttcgccgtcagagccagaatggctgagcctagctttggcggcttttggagcgcttggagcgagccagttagcctgctgacacctagcgatctggaccccgtggttatctctgttggctccatgggattgattatcagccttctctgtgtgtatttctggctggaacggacgatgccccgaattcccaccctgaagaacctagaggatcttgttactgaataccacgggaacttttcggcctggagtggtgtgtctaagggactggctgagagtctgcagccagactacagtgaacgactctgcctcgtcagtgagattcccccaaaaggaggggcccttggggaggggcctggggcctccccatgcaaccagcatagcccctactgggcccccccatgttacaccctaaagcctgaaacc

SEQ ID NO: 3 - protein, 601 aa, synthetic construct
  REGION 1..601: note = PEB amino acid sequence
RRKRGKPIPNPLLGLDSTSGSGATNFSLLKQAGDVEENPGPDHLGASLWPQVGSLCLLLAGAAWAPPPNLPDPKFESKAALLAARGPEELLCFTERLEDLVCFWEEAASAGVGPGNYSFSYQLEDEPWKLCRLHQAPTARGAVRFWCSLPTADTSSFVPLELRVTAASGAPRYHRVIHINEVVLLDAPVGLVARLADESGHVVLRWLPPPETPMTSHIRYEVDVSAGNGAGSVQRVEILEGRTECVLSNLRGRTRYTFAVRARMAEPSFGGFWSAWSEPVSLLTPSDLDPIPWLGHLLVGLSGAFGFIILVYLLINCRNTGPWLKKVLKCNTPDPSKFFSQLSSEHGGDVQKWLSSPFPSSSFSPGGLAPEISPLEVLERDKVTQLLLQQDKVPEPASLSSNHSLTSCFTNQGYFFFHLPDALEIEACQVYFTYDPYSEEDPDEGVAGAPTGSSPQPLQPLSGEDDAYCTFPSRDDLLLFSPSLLGGPSPPSTAPGGSGAGEERMPPSLQERVPRDWDPQPLGPPTPGVPDLVDFQPPPELVLREAGEEVPDAGPREGVSFPWSRPPGQGEFRALNARLPLNTDAYLSLQELQGQDPTHLV

SEQ ID NO: 4 - DNA, 1806 bp, synthetic construct
  misc_feature 1..1806: note = PEB nucleic acid sequence
  source 1..1806: mol_type = other DNA
agaagaaagcgcggaaagcctattccaaatccactcctcggcctggacagcacatctggatctggcgccaccaacttcagtctgctgaaacaggccggcgacgtcgaggaaaatcccgggccagatcatctcggagccagtctctggccacaagtcggaagcctgtgtttgttgctggctggtgcagcatgggccccaccaccaaatctccctgatccaaagtttgagtccaaagctgccctgctggccgcaagaggtcccgaagaactcctgtgttttacagagcggcttgaggatctcgtctgtttttgggaagaagccgcctccgctggcgtcggacccggcaattattcctttagctatcagctcgaggacgagccttggaaactgtgtcggctccaccaggctccaactgcaagaggcgccgttagattctggtgctctctgccaaccgccgataccagctcctttgtgcccctcgagcttagagtgactgctgctagcggagccccacggtatcatcgggtcatccatatcaatgaagtcgtcctgctggacgctcccgtgggacttgtcgctagactggctgacgaaagcggccacgttgtcctcagatggctcccacctcctgaaactcccatgacctctcacattcgctatgaagtggatgtctccgcaggcaacggtgccggaagcgttcagagagtcgagattctcgagggcagaacagagtgtgtgctgtctaacctgcggggcagaaccagatacacatttgctgtgcgcgccaggatggccgaaccttccttcggtggattttggagtgcttggagtgaacccgtgtctctgctgaccccttccgacctcgatcctattccgtggctcggccacctcctcgtgggcctcagcggggcttttggcttcatcatcttagtgtacttgctgatcaactgcaggaacaccgggccatggctgaagaaggtcctgaagtgtaacaccccagacccctcgaagttcttttcccagctgagctcagagcatggaggagacgtccagaagtggctctcttcgcccttcccctcatcgtccttcagccctggcggcctggcacctgagatctcgccactagaagtgctggagagggacaaggtgacgcagctgctcctgcagcaggacaaggtgcctgagcccgcatccttaagcagcaaccactcgctgaccagctgcttcaccaaccagggttacttcttcttccacctcccggatgccttggagatagaggcctgccaggtgtactttacttacgacccctactcagaggaagaccctgatgagggtgtggccggggcacccacagggtcttccccccaacccctgcagcctctgtcaggggaggacgacgcctactgcaccttcccctccagggatgacctgctgctcttctcccccagtctcctcggtggccccagccccccaagcactgcccctgggggcagtggggccggtgaagagaggatgcccccttctttgcaagaaagagtccccagagactgggacccccagcccctggggcctcccaccccaggagtcccagacctggtggattttcagccaccccctgagctggtgctgcgagaggctggggaggaggtccctgacgctggccccagggagggagtcagtttcccctggtccaggcctcctgggcagggggagttcagggcccttaatgctcgcctgcccctgaacactgatgcctacttgtccctccaagaactccagggtcaggacccaactcacttggtgtag

SEQ ID NO: 5 - protein, 997 aa, synthetic construct
  REGION 1..997: note = TEGPEB amino acid sequence
RAKRGKPIPNPLLGLDSTSGSGEGRGSLLTCGDVEENPGPDHLGASLWPQVGSLCLLLAGAAWAPPPNLPDPKFESKAALLAARGPEELLCFTERLEDLVCFWEEAASAGVGPGNYSFSYQLEDEPWKLCRLHQAPTARGAVRFWCSLPTADTSSFVPLELRVTAASGAPRYHRVIHINEVVLLDAPVGLVARLADESGHVVLRWLPPPETPMTSHIRYEVDVSAGNGAGSVQRVEILEGRTECVLSNLRGRTRYTFAVRARMAEPSFGGFWSAWSEPVSLLTPSDLDPVVISVGSMGLIISLLCVYFWLERTMPRIPTLKNLEDLVTEYHGNFSAWSGVSKGLAESLQPDYSERLCLVSEIPPKGGALGEGPGASPCNQHSPYWAPPCYTLKPETRRKRGKPIPNPLLGLDSTSGSGATNFSLLKQAGDVEENPGPDHLGASLWPQVGSLCLLLAGAAWAPPPNLPDPKFESKAALLAARGPEELLCFTERLEDLVCFWEEAASAGVGPGNYSFSYQLEDEPWKLCRLHQAPTARGAVRFWCSLPTADTSSFVPLELRVTAASGAPRYHRVIHINEVVLLDAPVGLVARLADESGHVVLRWLPPPETPMTSHIRYEVDVSAGNGAGSVQRVEILEGRTECVLSNLRGRTRYTFAVRARMAEPSFGGFWSAWSEPVSLLTPSDLDPIPWLGHLLVGLSGAFGFIILVYLLINCRNTGPWLKKVLKCNTPDPSKFFSQLSSEHGGDVQKWLSSPFPSSSFSPGGLAPEISPLEVLERDKVTQLLLQQDKVPEPASLSSNHSLTSCFTNQGYFFFHLPDALEIEACQVYFTYDPYSEEDPDEGVAGAPTGSSPQPLQPLSGEDDAYCTFPSRDDLLLFSPSLLGGPSPPSTAPGGSGAGEERMPPSLQERVPRDWDPQPLGPPTPGVPDLVDFQPPPELVLREAGEEVPDAGPREGVSFPWSRPPGQGEFRALNARLPLNTDAYLSLQELQGQDPTHLV

SEQ ID NO: 6 - DNA, 2994 bp, synthetic construct
  misc_feature 1..2994: note = TEGPEB nucleic acid sequence
  source 1..2994: mol_type = other DNA
agggccaagaggggcaagcccattcctaatcctctgctgggcctcgatagcacaagcggcagcggagaaggcagaggctctctgcttacatgcggcgacgtggaagagaaccccggacctgatcacctgggcgcttctctgtggcctcaagtgggatctctgtgtctgctgcttgctggcgctgcttgggctcctcctcctaatctgcccgatcctaagttcgagagcaaggccgctctgctggctgctagaggacctgaggaactgctgtgcttcaccgagagactcgaggacctcgtgtgcttctgggaagaagctgcttctgccggcgttggccctggcaattacagcttcagctaccagctggaagatgagccctggaagctgtgcagactgcatcaggcccctacagctagaggcgctgtgcggttttggtgtagcctgcctacagccgacaccagcagcttcgtgcctctggaactgagagtgacagccgcttctggcgcccctagataccacagagtgatccacatcaacgaggtggtgctgctggatgcccctgttggactggttgccagactggccgatgagtctggacatgtggtgctgagatggctgcctcctccagagacacctatgaccagccacatcagatacgaggtggacgtgtccgccggaaatggcgctggatctgtgcagagagtggaaatcctggaaggccggaccgagtgcgtgctgagcaatctgagaggcagaacccggtacaccttcgccgtcagagccagaatggctgagcctagctttggcggcttttggagcgcttggagcgagccagttagcctgctgacacctagcgatctggaccccgtggttatctctgttggctccatgggattgattatcagccttctctgtgtgtatttctggctggaacggacgatgccccgaattcccaccctgaagaacctagaggatcttgttactgaataccacgggaacttttcggcctggagtggtgtgtctaagggactggctgagagtctgcagccagactacagtgaacgactctgcctcgtcagtgagattcccccaaaaggaggggcccttggggaggggcctggggcctccccatgcaaccagcatagcccctactgggcccccccatgttacaccctaaagcctgaaaccagaagaaagcgcggaaagcctattccaaatccactcctcggcctggacagcacatctggatctggcgccaccaacttcagtctgctgaaacaggccggcgacgtcgaggaaaatcccgggccagatcatctcggagccagtctctggccacaagtcggaagcctgtgtttgttgctggctggtgcagcatgggccccaccaccaaatctccctgatccaaagtttgagtccaaagctgccctgctggccgcaagaggtcccgaagaactcctgtgttttacagagcggcttgaggatctcgtctgtttttgggaagaagccgcctccgctggcgtcggacccggcaattattcctttagctatcagctcgaggacgagccttggaaactgtgtcggctccaccaggctccaactgcaagaggcgccgttagattctggtgctctctgccaaccgccgataccagctcctttgtgcccctcgagcttagagtgactgctgctagcggagccccacggtatcatcgggtcatccatatcaatgaagtcgtcctgctggacgctcccgtgggacttgtcgctagactggctgacgaaagcggccacgttgtcctcagatggctcccacctcctgaaactcccatgacctctcacattcgctatgaagtggatgtctccgcaggcaacggtgccggaagcgttcagagagtcgagattctcgagggcagaacagagtgtgtgctgtctaacctgcggggcagaaccagatacacatttgctgtgcgcgccaggatggccgaaccttccttcggtggattttggagtgcttggagtgaacccgtgtctctgctgaccccttccgacctcgatcctattccgtggctcggccacctcctcgtgggcctcagcggggcttttggcttcatcatcttagtgtacttgctgatcaactgcaggaacaccgggccatggctgaagaaggtcctgaagtgtaacaccccagacccctcgaagttcttttcccagctgagctcagagcatggaggagacgtccagaagtggctctcttcgcccttcccctcatcgtccttcagccctggcggcctggcacctgagatctcgccactagaagtgctggagagggacaaggtgacgcagctgctcctgcagcaggacaaggtgcctgagcccgcatccttaagcagcaaccactcgctgaccagctgcttcaccaaccagggttacttcttcttccacctcccggatgccttggagatagaggcctgccaggtgtactttacttacgacccctactcagaggaagaccctgatgagggtgtggccggggcacccacagggtcttccccccaacccctgcagcctctgtcaggggaggacgacgcctactgcaccttcccctccagggatgacctgctgctcttctcccccagtctcctcggtggccccagccccccaagcactgcccctgggggcagtggggccggtgaagagaggatgcccccttctttgcaagaaagagtccccagagactgggacccccagcccctggggcctcccaccccaggagtcccagacctggtggattttcagccaccccctgagctggtgctgcgagaggctggggaggaggtccctgacgctggccccagggagggagtcagtttcccctggtccaggcctcctgggcagggggagttcagggcccttaatgctcgcctgcccctgaacactgatgcctacttgtccctccaagaactccagggtcaggacccaactcacttggtgtag

SEQ ID NO: 7 - DNA, 27 bp, synthetic construct
  misc_feature 1..27: note = pEX-V_InfRev primer
  source 1..27: mol_type = other DNA
atgccgtgagcacaaaagcgaccatag

SEQ ID NO: 8 - DNA, 26 bp, synthetic construct
  misc_feature 1..26: note = pEX-V_InfFwd primer
  source 1..26: mol_type = other DNA
agtcagtggatacgccaaatgccttc

SEQ ID NO: 9 - DNA, 41 bp, synthetic construct
  misc_feature 1..41: note = TSRG1_pEXInfFwd primer
  source 1..41: mol_type = other DNA
ttgtgctcacggcatagggccaagaggggcaagcccattcc

SEQ ID NO: 10 - DNA, 34 bp, synthetic construct
  misc_feature 1..34: note = TSRG1_pEXInfRev primer
  source 1..34: mol_type = other DNA
tccgcgctttcttctggtttcaggctttagggtg

SEQ ID NO: 11 - DNA, 34 bp, synthetic construct
  misc_feature 1..34: note = PSRG2_pEXInfFwd primer
  source 1..34: mol_type = other DNA
agaagaaagcgcggaaagcctattccaaatccac

SEQ ID NO: 12 - DNA, 39 bp, synthetic construct
  misc_feature 1..39: note = PSRG2_pEXInfRev primer
  source 1..39: mol_type = other DNA
gcgtatccactgactctacaccaagtgagttgggtcctg

SEQ ID NO: 13 - protein, 1228 aa, synthetic construct
  REGION 1..1228: note = ZG-SRG_YYY amino acid sequence
MAQSKHGLTKEMTMKYRMEGCVDGHKFVITGEGIGYPFKGKQAINLCVVEGGPLPFAEDILSAAFMYGNRVFTEYPQDIVDYFKNSCPAGYTWDRSFLFEDGAVCICNADITVSVEENCMYHESKFYGVNFPADGPVMKKMTDNWEPSCEKIIPVPKQGILKGDVSMYLLLKDGGRLRCQFDTVYKAKSVPRKMPDWHFIQHKLTREDRSDAKNQKWHLTEHAIASGSALPRAKRGKPIPNPLLGLDSTSGSGEGRGSLLTCGDVEENPGPDHLGASLWPQVGSLCLLLAGAAWAPPPNLPDPKFESKAALLAARGPEELLCFTERLEDLVCFWEEAASAGVGPGNYSFSYQLEDEPWKLCRLHQAPTARGAVRFWCSLPTADTSSFVPLELRVTAASGAPRYHRVIHINEVVLLDAPVGLVARLADESGHVVLRWLPPPETPMTSHIRYEVDVSAGNGAGSVQRVEILEGRTECVLSNLRGRTRYTFAVRARMAEPSFGGFWSAWSEPVSLLTPSDLDPVVISVGSMGLIISLLCVYFWLERTMPRIPTLKNLEDLVTEYHGNFSAWSGVSKGLAESLQPDYSERLCLVSEIPPKGGALGEGPGASPCNQHSPYWAPPCYTLKPETRRKRGKPIPNPLLGLDSTSGSGATNFSLLKQAGDVEENPGPDHLGASLWPQVGSLCLLLAGAAWAPPPNLPDPKFESKAALLAARGPEELLCFTERLEDLVCFWEEAASAGVGPGNYSFSYQLEDEPWKLCRLHQAPTARGAVRFWCSLPTADTSSFVPLELRVTAASGAPRYHRVIHINEVVLLDAPVGLVARLADESGHVVLRWLPPPETPMTSHIRYEVDVSAGNGAGSVQRVEILEGRTECVLSNLRGRTRYTFAVRARMAEPSFGGFWSAWSEPVSLLTPSDLDPIPWLGHLLVGLSGAFGFIILVYLLINCRNTGPWLKKVLKCNTPDPSKFFSQLSSEHGGDVQKWLSSPFPSSSFSPGGLAPEISPLEVLERDKVTQLLLQQDKVPEPASLSSNHSLTSCFTNQGYFFFHLPDALEIEACQVYFTYDPYSEEDPDEGVAGAPTGSSPQPLQPLSGEDDAYCTFPSRDDLLLFSPSLLGGPSPPSTAPGGSGAGEERMPPSLQERVPRDWDPQPLGPPTPGVPDLVDFQPPPELVLREAGEEVPDAGPREGVSFPWSRPPGQGEFRALNARLPLNTDAYLSLQELQGQDPTHLV

SEQ ID NO: 14 - DNA, 3687 bp, synthetic construct
  misc_feature 1..3687: note = ZG-SRG_YYY nucleic acid sequence
  source 1..3687: mol_type = other DNA
atggcccagtccaagcacggcctgaccaaggagatgaccatgaagtaccgcatggagggctgcgtggacggccacaagttcgtgatcaccggcgagggcatcggctaccccttcaagggcaagcaggccatcaacctgtgcgtggtggagggcggccccttgcccttcgccgaggacatcttgtccgccgccttcatgtacggcaaccgcgtgttcaccgagtacccccaggacatcgtcgactacttcaagaactcctgccccgccggctacacctgggaccgctccttcctgttcgaggacggcgccgtgtgcatctgcaacgccgacatcaccgtgagcgtggaggagaactgcatgtaccacgagtccaagttctacggcgtgaacttccccgccgacggccccgtgatgaagaagatgaccgacaactgggagccctcctgcgagaagatcatccccgtgcccaagcagggcatcttgaagggcgacgtgagcatgtacctgctgctgaaggacggtggccgcttgcgctgccagttcgacaccgtgtacaaggccaagtccgtgccccgcaagatgcccgactggcacttcatccagcacaagctgacccgcgaggaccgcagcgacgccaagaaccagaagtggcacctgaccgagcacgccatcgcctccggctccgccttgcccagggccaagaggggcaagcccattcctaatcctctgctgggcctcgatagcacaagcggcagcggagaaggcagaggctctctgcttacatgcggcgacgtggaagagaaccccggacctgatcacctgggcgcttctctgtggcctcaagtgggatctctgtgtctgctgcttgctggcgctgcttgggctcctcctcctaatctgcccgatcctaagttcgagagcaaggccgctctgctggctgctagaggacctgaggaactgctgtgcttcaccgagagactcgaggacctcgtgtgcttctgggaagaagctgcttctgccggcgttggccctggcaattacagcttcagctaccagctggaagatgagccctggaagctgtgcagactgcatcaggcccctacagctagaggcgctgtgcggttttggtgtagcctgcctacagccgacaccagcagcttcgtgcctctggaactgagagtgacagccgcttctggcgcccctagataccacagagtgatccacatcaacgaggtggtgctgctggatgcccctgttggactggttgccagactggccgatgagtctggacatgtggtgctgagatggctgcctcctccagagacacctatgaccagccacatcagatacgaggtggacgtgtccgccggaaatggcgctggatctgtgcagagagtggaaatcctggaaggccggaccgagtgcgtgctgagcaatctgagaggcagaacccggtacaccttcgccgtcagagccagaatggctgagcctagctttggcggcttttggagcgcttggagcgagccagttagcctgctgacacctagcgatctggaccccgtggttatctctgttggctccatgggattgattatcagccttctctgtgtgtatttctggctggaacggacgatgccccgaattcccaccctgaagaacctagaggatcttgttactgaataccacgggaacttttcggcctggagtggtgtgtctaagggactggctgagagtctgcagccagactacagtgaacgactctgcctcgtcagtgagattcccccaaaaggaggggcccttggggaggggcctggggcctccccatgcaaccagcatagcccctactgggcccccccatgttacaccctaaagcctgaaaccagaagaaagcgcggaaagcctattccaaatccactcctcggcctggacagcacatctggatctggcgccaccaacttcagtctgctgaaacaggccggcgacgtcgaggaaaatcccgggccagatcatctcggagccagtctctggccacaagtcggaagcctgtgtttgttgctggctggtgcagcatgggccccaccaccaaatctccctgatccaaagtttgagtccaaagctgccctgctggccgcaagaggtcccgaagaactcctgtgttttacagagcggcttgaggatctcgtctgtttttgggaagaagccgcctccgctggcgtcggacccggcaattattcctttagctatcagctcgaggacgagccttggaaactgtgtcggctccaccaggctccaactgcaagaggcgccgttagattctggtgctctctgccaaccgccgataccagctcctttgtgcccctcgagcttagagtgactgctgctagcggagccccacggtatcatcgggtcatccatatcaatgaagtcgtcctgctggacgctcccgtgggacttgtcgctagactggctgacgaaagcggccacgttgtcctcagatggctcccacctcctgaaactcccatgacctctcacattcgctatgaagtggatgtctccgcaggcaacggtgccggaagcgttcagagagtcgagattctcgagggcagaacagagtgtgtgctgtctaacctgcggggcagaaccagatacacatttgctgtgcgcgccaggatggccgaaccttccttcggtggattttggagtgcttggagtgaacccgtgtctctgctgaccccttccgacctcgatcctattccgtggctcggccacctcctcgtgggcctcagcggggcttttggcttcatcatcttagtgtacttgctgatcaactgcaggaacaccgggccatggctgaagaaggtcctgaagtgtaacaccccagacccctcgaagttcttttcccagctgagctcagagcatggaggagacgtccagaagtggctctcttcgcccttcccctcatcgtccttcagccctggcggcctggcacctgagatctcgccactagaagtgctggagagggacaaggtgacgcagctgctcctgcagcaggacaaggtgcctgagcccgcatccttaagcagcaaccactcgctgaccagctgcttcaccaaccagggttacttcttcttccacctcccggatgccttggagatagaggcctgccaggtgtactttacttacgacccctactcagaggaagaccctgatgagggtgtggccggggcacccacagggtcttccccccaacccctgcagcctctgtcaggggaggacgacgcctactgcaccttcccctccagggatgacctgctgctcttctcccccagtctcctcggtggccccagccccccaagcactgcccctgggggcagtggggccggtgaagagaggatgcccccttctttgcaagaaagagtccccagagactgggacccccagcccctggggcctcccaccccaggagtcccagacctggtggattttcagccaccccctgagctggtgctgcgagaggctggggaggaggtccctgacgctggccccagggagggagtcagtttcccctggtccaggcctcctgggcagggggagttcagggcccttaatgctcgcctgcccctgaacactgatgcctacttgtccctccaagaactccagggtcaggacccaactcacttggtgtag

SEQ ID NO: 15 - DNA, 47 bp, synthetic construct
  misc_feature 1..47: note = ZGSRG-ZG_M5InfFwd primer
  source 1..47: mol_type = other DNA
gagctcggatctcacgtgccaccatggcccagtccaagcacggcctg

SEQ ID NO: 16 - DNA, 34 bp, synthetic construct
  misc_feature 1..34: note = ZGSRG-ZG_M5InfRev primer
  source 1..34: mol_type = other DNA
gcccctcttggccctgggcaaggcggagccggag

SEQ ID NO: 17 - DNA, 34 bp, synthetic construct
  misc_feature 1..34: note = ZGSRG-SRG_M5InfFwd primer
  source 1..34: mol_type = other DNA
agggccaagaggggcaagcccattcctaatcctc

SEQ ID NO: 18 - DNA, 38 bp, synthetic construct
  misc_feature 1..38: note = ZGSRG-SRG_M5InfRev primer
  source 1..38: mol_type = other DNA
taacgtcgacggatccctacaccaagtgagttgggtcc

SEQ ID NO: 19 - protein, 1228 aa, synthetic construct
  REGION 1..1228: note = ZG-SRG_FYY amino acid sequence
MAQSKHGLTKEMTMKYRMEGCVDGHKFVITGEGIGYPFKGKQAINLCVVEGGPLPFAEDILSAAFMYGNRVFTEYPQDIVDYFKNSCPAGYTWDRSFLFEDGAVCICNADITVSVEENCMYHESKFYGVNFPADGPVMKKMTDNWEPSCEKIIPVPKQGILKGDVSMYLLLKDGGRLRCQFDTVYKAKSVPRKMPDWHFIQHKLTREDRSDAKNQKWHLTEHAIASGSALPRAKRGKPIPNPLLGLDSTSGSGEGRGSLLTCGDVEENPGPDHLGASLWPQVGSLCLLLAGAAWAPPPNLPDPKFESKAALLAARGPEELLCFTERLEDLVCFWEEAASAGVGPGNYSFSYQLEDEPWKLCRLHQAPTARGAVRFWCSLPTADTSSFVPLELRVTAASGAPRYHRVIHINEVVLLDAPVGLVARLADESGHVVLRWLPPPETPMTSHIRYEVDVSAGNGAGSVQRVEILEGRTECVLSNLRGRTRYTFAVRARMAEPSFGGFWSAWSEPVSLLTPSDLDPVVISVGSMGLIISLLCVYFWLERTMPRIPTLKNLEDLVTEYHGNFSAWSGVSKGLAESLQPDYSERLCLVSEIPPKGGALGEGPGASPCNQHSPYWAPPCYTLKPETRRKRGKPIPNPLLGLDSTSGSGATNFSLLKQAGDVEENPGPDHLGASLWPQVGSLCLLLAGAAWAPPPNLPDPKFESKAALLAARGPEELLCFTERLEDLVCFWEEAASAGVGPGNYSFSYQLEDEPWKLCRLHQAPTARGAVRFWCSLPTADTSSFVPLELRVTAASGAPRYHRVIHINEVVLLDAPVGLVARLADESGHVVLRWLPPPETPMTSHIRYEVDVSAGNGAGSVQRVEILEGRTECVLSNLRGRTRYTFAVRARMAEPSFGGFWSAWSEPVSLLTPSDLDPIPWLGHLLVGLSGAFGFIILVYLLINCRNTGPWLKKVLKCNTPDPSKFFSQLSSEHGGDVQKWLSSPFPSSSFSPGGLAPEISPLEVLERDKVTQLLLQQDKVPEPASLSSNHSLTSCFTNQGYFFFHLPDALEIEACQVFFTYDPYSEEDPDEGVAGAPTGSSPQPLQPLSGEDDAYCTFPSRDDLLLFSPSLLGGPSPPSTAPGGSGAGEERMPPSLQERVPRDWDPQPLGPPTPGVPDLVDFQPPPELVLREAGEEVPDAGPREGVSFPWSRPPGQGEFRALNARLPLNTDAYLSLQELQGQDPTHLV

SEQ ID NO: 20 - DNA, 3687 bp, synthetic construct
  misc_feature 1..3687: note = ZG-SRG_FYY nucleic acid sequence
  source 1..3687: mol_type = other DNA
atggcccagtccaagcacggcctgaccaaggagatgaccatgaagtaccgcatggagggctgcgtggacggccacaagttcgtgatcaccggcgagggcatcggctaccccttcaagggcaagcaggccatcaacctgtgcgtggtggagggcggccccttgcccttcgccgaggacatcttgtccgccgccttcatgtacggcaaccgcgtgttcaccgagtacccccaggacatcgtcgactacttcaagaactcctgccccgccggctacacctgggaccgctccttcctgttcgaggacggcgccgtgtgcatctgcaacgccgacatcaccgtgagcgtggaggagaactgcatgtaccacgagtccaagttctacggcgtgaacttccccgccgacggccccgtgatgaagaagatgaccgacaactgggagccctcctgcgagaagatcatccccgtgcccaagcagggcatcttgaagggcgacgtgagcatgtacctgctgctgaaggacggtggccgcttgcgctgccagttcgacaccgtgtacaaggccaagtccgtgccccgcaagatgcccgactggcacttcatccagcacaagctgacccgcgaggaccgcagcgacgccaagaaccagaagtggcacctgaccgagcacgccatcgcctccggctccgccttgcccagggccaagaggggcaagcccattcctaatcctctgctgggcctcgatagcacaagcggcagcggagaaggcagaggctctctgcttacatgcggcgacgtggaagagaaccccggacctgatcacctgggcgcttctctgtggcctcaagtgggatctctgtgtctgctgcttgctggcgctgcttgggctcctcctcctaatctgcccgatcctaagttcgagagcaaggccgctctgctggctgctagaggacctgaggaactgctgtgcttcaccgagagactcgaggacctcgtgtgcttctgggaagaagctgcttctgccggcgttggccctggcaattacagcttcagctaccagctggaagatgagccctggaagctgtgcagactgcatcaggcccctacagctagaggcgctgtgcggttttggtgtagcctgcctacagccgacaccagcagcttcgtgcctctggaactgagagtgacagccgcttctggcgcccctagataccacagagtgatccacatcaacgaggtggtgctgctggatgcccctgttggactggttgccagactggccgatgagtctggacatgtggtgctgagatggctgcctcctccagagacacctatgaccagccacatcagatacgaggtggacgtgtccgccggaaatggcgctggatctgtgcagagagtggaaatcctggaaggccggaccgagtgcgtgctgagcaatctgagaggcagaacccggtacaccttcgccgtcagagccagaatggctgagcctagctttggcggcttttggagcgcttggagcgagccagttagcctgctgacacctagcgatctggaccccgtggttatctctgttggctccatgggattgattatcagccttctctgtgtgtatttctggctggaacggacgatgccccgaattcccaccctgaagaacctagaggatcttgttactgaataccacgggaacttttcggcctggagtggtgtgtctaagggactggctgagagtctgcagccagactacagtgaacgactctgcctcgtcagtgagattcccccaaaaggaggggcccttggggaggggcctggggcctccccatgcaaccagcatagcccctactgggcccccccatgttacaccctaaagcctgaaaccagaagaaagcgcggaaagcctattccaaatccactcctcggcctggacagcacatctggatctggcgccaccaacttcagtctgctgaaacaggccggcgacgtcgaggaaaatcccgggccagatcatctcggagccagtctctggccacaagtcggaagcctgtgtttgttgctggctggtgcagcatgggccccaccaccaaatctccctgatccaaagtttgagtccaaagctgccctgctggccgcaagaggtcccgaagaactcctgtgttttacagagcggcttgaggatctcgtctgtttttgggaagaagccgcctccgctggcgtcggacccggcaattattcctttagctatcagctcgaggacgagccttggaaactgtgtcggctccaccaggctccaactgcaagaggcgccgttagattctggtgctctctgccaaccgccgataccagctcctttgtgcccctcgagcttagagtgactgctgctagcggagccccacggtatcatcgggtcatccatatcaatgaagtcgtcctgctggacgctcccgtgggacttgtcgctagactggctgacgaaagcggccacgttgtcctcagatggctcccacctcctgaaactcccatgacctctcacattcgctatgaagtggatgtctccgcaggcaacggtgccggaagcgttcagagagtcgagattctcgagggcagaacagagtgtgtgctgtctaacctgcggggcagaaccagatacacatttgctgtgcgcgccaggatggccgaaccttccttcggtggattttggagtgcttggagtgaacccgtgtctctgctgaccccttccgacctcgatcctattccgtggctcggccacctcctcgtgggcctcagcggggcttttggcttcatcatcttagtgtacttgctgatcaactgcaggaacaccgggccatggctgaagaaggtcctgaagtgtaacaccccagacccctcgaagttcttttcccagctgagctcagagcatggaggagacgtccagaagtggctctcttcgcccttcccctcatcgtccttcagccctggcggcctggcacctgagatctcgccactagaagtgctggagagggacaaggtgacgcagctgctcctgcagcaggacaaggtgcctgagcccgcatccttaagcagcaaccactcgctgaccagctgcttcaccaaccagggttacttcttcttccacctcccggatgccttggagatagaggcctgccaggtgttctttacttacgacccctactcagaggaagaccctgatgagggtgtggccggggcacccacagggtcttccccccaacccctgcagcctctgtcaggggaggacgacgcctactgcaccttcccctccagggatgacctgctgctcttctcccccagtctcctcggtggccccagccccccaagcactgcccctgggggcagtggggccggtgaagagaggatgcccccttctttgcaagaaagagtccccagagactgggacccccagcccctggggcctcccaccccaggagtcccagacctggtggattttcagccaccccctgagctggtgctgcgagaggctggggaggaggtccctgacgctggccccagggagggagtcagtttcccctggtccaggcctcctgggcagggggagttcagggcccttaatgctcgcctgcccctgaacactgatgcctacttgtccctccaagaactccagggtcaggacccaactcacttggtgtag

SEQ ID NO: 21 - DNA, 23 bp, synthetic construct
  misc_feature 1..23: note = FYYmut_Rev primer
  source 1..23: mol_type = other DNA
acacctggcaggcctctatctcc

SEQ ID NO: 22 - DNA, 35 bp, synthetic construct
  misc_feature 1..35: note = FYYmut_Fwd primer
  source 1..35: mol_type = other DNA
aggcctgccaggtgtactttactttcgacccctac

SEQ ID NO: 23 - protein, 1228 aa, synthetic construct
  REGION 1..1228: note = ZG-SRG_YFY amino acid sequence
MAQSKHGLTKEMTMKYRMEGCVDGHKFVITGEGIGYPFKGKQAINLCVVEGGPLPFAEDILSAAFMYGNRVFTEYPQDIVDYFKNSCPAGYTWDRSFLFEDGAVCICNADITVSVEENCMYHESKFYGVNFPADGPVMKKMTDNWEPSCEKIIPVPKQGILKGDVSMYLLLKDGGRLRCQFDTVYKAKSVPRKMPDWHFIQHKLTREDRSDAKNQKWHLTEHAIASGSALPRAKRGKPIPNPLLGLDSTSGSGEGRGSLLTCGDVEENPGPDHLGASLWPQVGSLCLLLAGAAWAPPPNLPDPKFESKAALLAARGPEELLCFTERLEDLVCFWEEAASAGVGPGNYSFSYQLEDEPWKLCRLHQAPTARGAVRFWCSLPTADTSSFVPLELRVTAASGAPRYHRVIHINEVVLLDAPVGLVARLADESGHVVLRWLPPPETPMTSHIRYEVDVSAGNGAGSVQRVEILEGRTECVLSNLRGRTRYTFAVRARMAEPSFGGFWSAWSEPVSLLTPSDLDPVVISVGSMGLIISLLCVYFWLERTMPRIPTLKNLEDLVTEYHGNFSAWSGVSKGLAESLQPDYSERLCLVSEIPPKGGALGEGPGASPCNQHSPYWAPPCYTLKPETRRKRGKPIPNPLLGLDSTSGSGATNFSLLKQAGDVEENPGPDHLGASLWPQVGSLCLLLAGAAWAPPPNLPDPKFESKAALLAARGPEELLCFTERLEDLVCFWEEAASAGVGPGNYSFSYQLEDEPWKLCRLHQAPTARGAVRFWCSLPTADTSSFVPLELRVTAASGAPRYHRVIHINEVVLLDAPVGLVARLADESGHVVLRWLPPPETPMTSHIRYEVDVSAGNGAGSVQRVEILEGRTECVLSNLRGRTRYTFAVRARMAEPSFGGFWSAWSEPVSLLTPSDLDPIPWLGHLLVGLSGAFGFIILVYLLINCRNTGPWLKKVLKCNTPDPSKFFSQLSSEHGGDVQKWLSSPFPSSSFSPGGLAPEISPLEVLERDKVTQLLLQQDKVPEPASLSSNHSLTSCFTNQGYFFFHLPDALEIEACQVYFTFDPYSEEDPDEGVAGAPTGSSPQPLQPLSGEDDAYCTFPSRDDLLLFSPSLLGGPSPPSTAPGGSGAGEERMPPSLQERVPRDWDPQPLGPPTPGVPDLVDFQPPPELVLREAGEEVPDAGPREGVSFPWSRPPGQGEFRALNARLPLNTDAYLSLQELQGQDPTHLV

SEQ ID NO: 24 - DNA, 3687 bp, synthetic construct
  misc_feature 1..3687: note = ZG-SRG_YFY nucleic acid sequence
  source 1..3687: mol_type = other DNA
atggcccagtccaagcacggcctgaccaaggagatgaccatgaagtaccgcatggagggctgcgtggacggccacaagttcgtgatcaccggcgagggcatcggctaccccttcaagggcaagcaggccatcaacctgtgcgtggtggagggcggccccttgcccttcgccgaggacatcttgtccgccgccttcatgtacggcaaccgcgtgttcaccgagtacccccaggacatcgtcgactacttcaagaactcctgccccgccggctacacctgggaccgctccttcctgttcgaggacggcgccgtgtgcatctgcaacgccgacatcaccgtgagcgtggaggagaactgcatgtaccacgagtccaagttctacggcgtgaacttccccgccgacggccccgtgatgaagaagatgaccgacaactgggagccctcctgcgagaagatcatccccgtgcccaagcagggcatcttgaagggcgacgtgagcatgtacctgctgctgaaggacggtggccgcttgcgctgccagttcgacaccgtgtacaaggccaagtccgtgccccgcaagatgcccgactggcacttcatccagcacaagctgacccgcgaggaccgcagcgacgccaagaaccagaagtggcacctgaccgagcacgccatcgcctccggctccgccttgcccagggccaagaggggcaagcccattcctaatcctctgctgggcctcgatagcacaagcggcagcggagaaggcagaggctctctgcttacatgcggcgacgtggaagagaaccccggacctgatcacctgggcgcttctctgtggcctcaagtgggatctctgtgtctgctgcttgctggcgctgcttgggctcctcctcctaatctgcccgatcctaagttcgagagcaaggccgctctgctggctgctagaggacctgaggaactgctgtgcttcaccgagagactcgaggacctcgtgtgcttctgggaagaagctgcttctgccggcgttggccctggcaattacagcttcagctaccagctggaagatgagccctggaagctgtgcagactgcatcaggcccctacagctagaggcgctgtgcggttttggtgtagcctgcctacagccgacaccagcagcttcgtgcctctggaactgagagtgacagccgcttctggcgcccctagataccacagagtgatccacatcaacgaggtggtgctgctggatgcccctgttggactggttgccagactggccgatgagtctggacatgtggtgctgagatggctgcctcctccagagacacctatgaccagccacatcagatacgaggtggacgtgtccgccggaaatggcgctggatctgtgcagagagtggaaatcctggaaggccggaccgagtgcgtgctgagcaatctgagaggcagaacccggtacaccttcgccgtcagagccagaatggctgagcctagctttggcggcttttggagcgcttggagcgagccagttagcctgctgacacctagcgatctggaccccgtggttatctctgttggctccatgggattgattatcagccttctctgtgtgtatttctggctggaacggacgatgccccgaattcccaccctgaagaacctagaggatcttgttactgaataccacgggaacttttcggcctggagtggtgtgtctaagggactggctgagagtctgcagccagactacagtgaacgactctgcctcgtcagtgagattcccccaaaaggaggggcccttggggaggggcctggggcctccccatgcaaccagcatagcccctactgggcccccccatgttacaccctaaagcctgaaaccagaagaaagcgcggaaagcctattccaaatccactcctcggcctggacagcacatctggatctggcgccaccaacttcagtctgctgaaacaggccggcgacgtcgaggaaaatcccgggccagatcatctcggagccagtctctggccacaagtcggaagcctgtgtttgttgctggctggtgcagcatgggccccaccaccaaatctccctgatccaaagtttgagtccaaagctgccctgctggccgcaagaggtcccgaagaactcctgtgttttacagagcggcttgaggatctcgtctgtttttgggaagaagccgcctccgctggcgtcggacccggcaattattcctttagctatcagctcgaggacgagccttggaaactgtgtcggctccaccaggctccaactgcaagaggcgccgttagattctggtgctctctgccaaccgccgataccagctcctttgtgcccctcgagcttagagtgactgctgctagcggagccccacggtatcatcgggtcatccatatcaatgaagtcgtcctgctggacgctcccgtgggacttgtcgctagactggctgacgaaagcggccacgttgtcctcagatggctcccacctcctgaaactcccatgacctctcacattcgctatgaagtggatgtctccgcaggcaacggtgccggaagcgttcagagagtcgagattctcgagggcagaacagagtgtgtgctgtctaacctgcggggcagaaccagatacacatttgctgtgcgcgccaggatggccgaaccttccttcggtggattttggagtgcttggagtgaacccgtgtctctgctgaccccttccgacctcgatcctattccgtggctcggccacctcctcgtgggcctcagcggggcttttggcttcatcatcttagtgtacttgctgatcaactgcaggaacaccgggccatggctgaagaaggtcctgaagtgtaacaccccagacccctcgaagttcttttcccagctgagctcagagcatggaggagacgtccagaagtggctctcttcgcccttcccctcatcgtccttcagccctggcggcctggcacctgagatctcgccactagaagtgctggagagggacaaggtgacgcagctgctcctgcagcaggacaaggtgcctgagcccgcatccttaagcagcaaccactcgctgaccagctgcttcaccaaccagggttacttcttcttccacctcccggatgccttggagatagaggcctgccaggtgtactttactttcgacccctactcagaggaagaccctgatgagggtgtggccggggcacccacagggtcttccccccaacccctgcagcctctgtcaggggaggacgacgcctactgcaccttcccctccagggatgacctgctgctcttctcccccagtctcctcggtggccccagccccccaagcactgcccctgggggcagtggggccggtgaagagaggatgcccccttctttgcaagaaagagtccccagagactgggacccccagcccctggggcctcccaccccaggagtcccagacctggtggattttcagccaccccctgagctggtgctgcgagaggctggggaggaggtccctgacgctggccccagggagggagtcagtttcccctggtccaggcctcctgggcagggggagttcagggcccttaatgctcgcctgcccctgaacactgatgcctacttgtccctccaagaactccagggtcaggacccaactcacttggtgtag

SEQ ID NO: 25 - DNA, 23 bp, synthetic construct
  misc_feature 1..23: note = YFYmut_Rev primer
  source 1..23: mol_type = other DNA
acacctggcaggcctctatctcc

SEQ ID NO: 26 - DNA, 35 bp, synthetic construct; identical to SEQ ID NO: 22
  misc_feature 1..35: note = YFYmut_Fwd primer
  source 1..35: mol_type = other DNA

SEQ ID NO: 27 - protein, 1228 aa, synthetic construct
  REGION 1..1228: note = ZG-SRG_YYF amino acid sequence
MAQSKHGLTKEMTMKYRMEGCVDGHKFVITGEGIGYPFKGKQAINLCVVEGGPLPFAEDILSAAFMYGNRVFTEYPQDIVDYFKNSCPAGYTWDRSFLFEDGAVCICNADITVSVEENCMYHESKFYGVNFPADGPVMKKMTDNWEPSCEKIIPVPKQGILKGDVSMYLLLKDGGRLRCQFDTVYKAKSVPRKMPDWHFIQHKLTREDRSDAKNQKWHLTEHAIASGSALPRAKRGKPIPNPLLGLDSTSGSGEGRGSLLTCGDVEENPGPDHLGASLWPQVGSLCLLLAGAAWAPPPNLPDPKFESKAALLAARGPEELLCFTERLEDLVCFWEEAASAGVGPGNYSFSYQLEDEPWKLCRLHQAPTARGAVRFWCSLPTADTSSFVPLELRVTAASGAPRYHRVIHINEVVLLDAPVGLVARLADESGHVVLRWLPPPETPMTSHIRYEVDVSAGNGAGSVQRVEILEGRTECVLSNLRGRTRYTFAVRARMAEPSFGGFWSAWSEPVSLLTPSDLDPVVISVGSMGLIISLLCVYFWLERTMPRIPTLKNLEDLVTEYHGNFSAWSGVSKGLAESLQPDYSERLCLVSEIPPKGGALGEGPGASPCNQHSPYWAPPCYTLKPETRRKRGKPIPNPLLGLDSTSGSGATNFSLLKQAGDVEENPGPDHLGASLWPQVGSLCLLLAGAAWAPPPNLPDPKFESKAALLAARGPEELLCFTERLEDLVCFWEEAASAGVGPGNYSFSYQLEDEPWKLCRLHQAPTARGAVRFWCSLPTADTSSFVPLELRVTAASGAPRYHRVIHINEVVLLDAPVGLVARLADESGHVVLRWLPPPETPMTSHIRYEVDVSAGNGAGSVQRVEILEGRTECVLSNLRGRTRYTFAVRARMAEPSFGGFWSAWSEPVSLLTPSDLDPIPWLGHLLVGLSGAFGFIILVYLLINCRNTGPWLKKVLKCNTPDPSKFFSQLSSEHGGDVQKWLSSPFPSSSFSPGGLAPEISPLEVLERDKVTQLLLQQDKVPEPASLSSNHSLTSCFTNQGYFFFHLPDALEIEACQVYFTYDPFSEEDPDEGVAGAPTGSSPQPLQPLSGEDDAYCTFPSRDDLLLFSPSLLGGPSPPSTAPGGSGAGEERMPPSLQERVPRDWDPQPLGPPTPGVPDLVDFQPPPELVLREAGEEVPDAGPREGVSFPWSRPPGQGEFRALNARLPLNTDAYLSLQELQGQDPTHLV

SEQ ID NO: 28 - DNA, 3687 bp, synthetic construct
  misc_feature 1..3687: note = ZG-SRG_YYF nucleic acid sequence
  source 1..3687: mol_type = other DNA
atggcccagtccaagcacggcctgaccaaggagatgaccatgaagtaccgcatggagggctgcgtggacggccacaagttcgtgatcaccggcgagggcatcggctaccccttcaagggcaagcaggccatcaacctgtgcgtggtggagggcggccccttgcccttcgccgaggacatcttgtccgccgccttcatgtacggcaaccgcgtgttcaccgagtacccccaggacatcgtcgactacttcaagaactcctgccccgccggctacacctgggaccgctccttcctgttcgaggacggcgccgtgtgcatctgcaacgccgacatcaccgtgagcgtggaggagaactgcatgtaccacgagtccaagttctacggcgtgaacttccccgccgacggccccgtgatgaagaagatgaccgacaactgggagccctcctgcgagaagatcatccccgtgcccaagcagggcatcttgaagggcgacgtgagcatgtacctgctgctgaaggacggtggccgcttgcgctgccagttcgacaccgtgtacaaggccaagtccgtgccccgcaagatgcccgactggcacttcatccagcacaagctgacccgcgaggaccgcagcgacgccaagaaccagaagtggcacctgaccgagcacgccatcgcctccggctccgccttgcccagggccaagaggggcaagcccattcctaatcctctgctgggcctcgatagcacaagcggcagcggagaaggcagaggctctctgcttacatgcggcgacgtggaagagaaccccggacctgatcacctgggcgcttctctgtggcctcaagtgggatctctgtgtctgctgcttgctggcgctgcttgggctcctcctcctaatctgcccgatcctaagttcgagagcaaggccgctctgctggctgctagaggacctgaggaactgctgtgcttcaccgagagactcgaggacctcgtgtgcttctgggaagaagctgcttctgccggcgttggccctggcaattacagcttcagctaccagctggaagatgagccctggaagctgtgcagactgcatcaggcccctacagctagaggcgctgtgcggttttggtgtagcctgcctacagccgacaccagcagcttcgtgcctctggaactgagagtgacagccgcttctggcgcccctagataccacagagtgatccacatcaacgaggtggtgctgctggatgcccctgttggactggttgccagactggccgatgagtctggacatgtggtgctgagatggctgcctcctccagagacacctatgaccagccacatcagatacgaggtggacgtgtccgccggaaatggcgctggatctgtgcagagagtggaaatcctggaaggccggaccgagtgcgtgctgagcaatctgagaggcagaacccggtacaccttcgccgtcagagccagaatggctgagcctagctttggcggcttttggagcgcttggagcgagccagttagcctgctgacacctagcgatctggaccccgtggttatctctgttggctccatgggattgattatcagccttctctgtgtgtatttctggctggaacggacgatgccccgaattcccaccctgaagaacctagaggatcttgttactgaataccacgggaacttttcggcctggagtggtgtgtctaagggactggctgagagtctgcagccagactacagtgaacgactctgcctcgtcagtgagattcccccaaaaggaggggcccttggggaggggcctggggcctccccatgcaaccagcatagcccctactgggcccccccatgttacaccctaaagcctgaaaccagaagaaagcgcggaaagcctattccaaatccactcctcggcctggacagcacatctggatctggcgccaccaacttcagtctgctgaaacaggccggcgacgtcgaggaaaatcccgggccagatcatctcggagccagtctctggccacaagtcggaagcctgtgtttgttgctggctggtgcagcatgggccccaccaccaaatctccctgatccaaagtttgagtccaaagctgccctgctggccgcaagaggtcccgaagaactcctgtgttttacagagcggcttgaggatctcgtctgtttttgggaagaagccgcctccgctggcgtcggacccggcaattattcctttagctatcagctcgaggacgagccttggaaactgtgtcggctccaccaggctccaactgcaagaggcgccgttagattctggtgctctctgccaaccgccgataccagctcctttgtgcccctcgagcttagagtgactgctgctagcggagccccacggtatcatcgggtcatccatatcaatgaagtcgtcctgctggacgctcccgtgggacttgtcgctagactggctgacgaaagcggccacgttgtcctcagatggctcccacctcctgaaactcccatgacctctcacattcgctatgaagtggatgtctccgcaggcaacggtgccggaagcgttcagagagtcgagattctcgagggcagaacagagtgtgtgctgtctaacctgcggggcagaaccagatacacatttgctgtgcgcgccaggatggccgaaccttccttcggtggattttggagtgcttggagtgaacccgtgtctctgctgaccccttccgacctcgatcctattccgtggctcggccacctcctcgtgggcctcagcggggcttttggcttcatcatcttagtgtacttgctgatcaactgcaggaacaccgggccatggctgaagaaggtcctgaagtgtaacaccccagacccctcgaagttcttttcccagctgagctcagagcatggaggagacgtccagaagtggctctcttcgcccttcccctcatcgtccttcagccctggcggcctggcacctgagatctcgccactagaagtgctggagagggacaaggtgacgcagctgctcctgcagcaggacaaggtgcctgagcccgcatccttaagcagcaaccactcgctgaccagctgcttcaccaaccagggttacttcttcttccacctcccggatgccttggagatagaggcctgccaggtgtactttacttacgaccccttctcagaggaagaccctgatgagggtgtggccggggcacccacagggtcttccccccaacccctgcagcctctgtcaggggaggacgacgcctactgcaccttcccctccagggatgacctgctgctcttctcccccagtctcctcggtggccccagccccccaagcactgcccctgggggcagtggggccggtgaagagaggatgcccccttctttgcaagaaagagtccccagagactgggacccccagcccctggggcctcccaccccaggagtcccagacctggtggattttcagccaccccctgagctggtgctgcgagaggctggggaggaggtccctgacgctggccccagggagggagtcagtttcccctggtccaggcctcctgggcagggggagttcagggcccttaatgctcgcctgcccctgaacactgatgcctacttgtccctccaagaactccagggtcaggacccaactcacttggtgtag

SEQ ID NO: 29 - DNA, 33 bp, synthetic construct
  misc_feature 1..33: note = YYFmut_Rev primer
  source 1..33: mol_type = other DNA
ggggtcgtaagtaaagtacacctggcaggcctc

SEQ ID NO: 30 - DNA, 34 bp, synthetic construct
  misc_feature 1..34: note = YYFmut_Fwd primer
  source 1..34: mol_type = other DNA
tttacttacgaccccttctcagaggaagaccctg

SEQ ID NO: 31 - protein, 1228 aa, synthetic construct
  REGION 1..1228: note = ZG-SRG_FFY amino acid sequence
MAQSKHGLTKEMTMKYRMEGCVDGHKFVITGEGIGYPFKGKQAINLCVVEGGPLPFAEDILSAAFMYGNRVFTEYPQDIVDYFKNSCPAGYTWDRSFLFEDGAVCICNADITVSVEENCMYHESKFYGVNFPADGPVMKKMTDNWEPSCEKIIPVPKQGILKGDVSMYLLLKDGGRLRCQFDTVYKAKSVPRKMPDWHFIQHKLTREDRSDAKNQKWHLTEHAIASGSALPRAKRGKPIPNPLLGLDSTSGSGEGRGSLLTCGDVEENPGPDHLGASLWPQVGSLCLLLAGAAWAPPPNLPDPKFESKAALLAARGPEELLCFTERLEDLVCFWEEAASAGVGPGNYSFSYQLEDEPWKLCRLHQAPTARGAVRFWCSLPTADTSSFVPLELRVTAASGAPRYHRVIHINEVVLLDAPVGLVARLADESGHVVLRWLPPPETPMTSHIRYEVDVSAGNGAGSVQRVEILEGRTECVLSNLRGRTRYTFAVRARMAEPSFGGFWSAWSEPVSLLTPSDLDPVVISVGSMGLIISLLCVYFWLERTMPRIPTLKNLEDLVTEYHGNFSAWSGVSKGLAESLQPDYSERLCLVSEIPPKGGALGEGPGASPCNQHSPYWAPPCYTLKPETRRKRGKPIPNPLLGLDSTSGSGATNFSLLKQAGDVEENPGPDHLGASLWPQVGSLCLLLAGAAWAPPPNLPDPKFESKAALLAARGPEELLCFTERLEDLVCFWEEAASAGVGPGNYSFSYQLEDEPWKLCRLHQAPTARGAVRFWCSLPTADTSSFVPLELRVTAASGAPRYHRVIHINEVVLLDAPVGLVARLADESGHVVLRWLPPPETPMTSHIRYEVDVSAGNGAGSVQRVEILEGRTECVLSNLRGRTRYTFAVRARMAEPSFGGFWSAWSEPVSLLTPSDLDPIPWLGHLLVGLSGAFGFIILVYLLINCRNTGPWLKKVLKCNTPDPSKFFSQLSSEHGGDVQKWLSSPFPSSSFSPGGLAPEISPLEVLERDKVTQLLLQQDKVPEPASLSSNHSLTSCFTNQGYFFFHLPDALEIEACQVFFTFDPYSEEDPDEGVAGAPTGSSPQPLQPLSGEDDAYCTFPSRDDLLLFSPSLLGGPSPPSTAPGGSGAGEERMPPSLQERVPRDWDPQPLGPPTPGVPDLVDFQPPPELVLREAGEEVPDAGPREGVSFPWSRPPGQGEFRALNARLPLNTDAYLSLQELQGQDPTHLV

SEQ ID NO: 32 - DNA, 3687 bp, synthetic construct
  misc_feature 1..3687: note = ZG-SRG_FFY nucleic acid sequence
  source 1..3687: mol_type = other DNA
atggcccagtccaagcacggcctgaccaaggagatgaccatgaagtaccgcatggagggctgcgtggacggccacaagttcgtgatcaccggcgagggcatcggctaccccttcaagggcaagcaggccatcaacctgtgcgtggtggagggcggccccttgcccttcgccgaggacatcttgtccgccgccttcatgtacggcaaccgcgtgttcaccgagtacccccaggacatcgtcgactacttcaagaactcctgccccgccggctacacctgggaccgctccttcctgttcgaggacggcgccgtgtgcatctgcaacgccgacatcaccgtgagcgtggaggagaactgcatgtaccacgagtccaagttctacggcgtgaacttccccgccgacggccccgtgatgaagaagatgaccgacaactgggagccctcctgcgagaagatcatccccgtgcccaagcagggcatcttgaagggcgacgtgagcatgtacctgctgctgaaggacggtggccgcttgcgctgccagttcgacaccgtgtacaaggccaagtccgtgccccgcaagatgcccgactggcacttcatccagcacaagctgacccgcgaggaccgcagcgacgccaagaaccagaagtggcacctgaccgagcacgccatcgcctccggctccgccttgcccagggccaagaggggcaagcccattcctaatcctctgctgggcctcgatagcacaagcggcagcggagaaggcagaggctctctgcttacatgcggcgacgtggaagagaaccccggacctgatcacctgggcgcttctctgtggcctcaagtgggatctctgtgtctgctgcttgctggcgctgcttgggctcctcctcctaatctgcccgatcctaagttcgagagcaaggccgctctgctggctgctagaggacctgaggaactgctgtgcttcaccgagagactcgaggacctcgtgtgcttctgggaagaagctgcttctgccggcgttggccctggcaattacagcttcagctaccagctggaagatgagccctggaagctgtgcagactgcatcaggcccctacagctagaggcgctgtgcggttttggtgtagcctgcctacagccgacaccagcagcttcgtgcctctggaactgagagtgacagccgcttctggcgcccctagataccacagagtgatccacatcaacgaggtggtgctgctggatgcccctgttggactggttgccagactggccgatgagtctggacatgtggtgctgagatggctgcctcctccagagacacctatgaccagccacatcagatacgaggtggacgtgtccgccggaaatggcgctggatctgtgcagagagtggaaatcctggaaggccggaccgagtgcgtgctgagcaatctgagaggcagaacccggtacaccttcgccgtcagagccagaatggctgagcctagctttggcggcttttggagcgcttggagcgagccagttagcctgctgacacctagcgatctggaccccgtggttatctctgttggctccatgggattgattatcagccttctctgtgtgtatttctggctggaacggacgatgccccgaattcccaccctgaagaacctagaggatcttgttactgaataccacgggaacttttcggcctggagtggtgtgtctaagggactggctgagagtctgcagccagactacagtgaacgactctgcctcgtcagtgagattcccccaaaaggaggggcccttggggaggggcctggggcctccccatgcaaccagcatagcccctactgggcccccccatgttacaccctaaagcctgaaaccagaagaaagcgcggaaagcctattccaaatccactcctcggcctggacagcacatctggatctggcgccaccaacttcagtctgctgaaacaggccggcgacgtcgaggaaaatcccgggccagatcatctcggagccagtctctggccacaagtcggaagcctgtgtttgttgctggctggtgcagcatgggccccaccaccaaatctccctgatccaaagtttgagtccaaagctgccctgctggccgcaagaggtcccgaagaactcctgtgttttacagagcggcttgaggatctcgtctgtttttgggaagaagccgcctccgctggcgtcggacccggcaattattcctttagctatcagctcgaggacgagccttggaaactgtgtcggctccaccaggctccaactgcaagaggcgccgttagattctggtgctctctgccaaccgccgataccagctcctttgtgcccctcgagcttagagtgactgctgctagcggagccccacggtatcatcgggtcatccatatcaatgaagtcgtcctgctggacgctcccgtgggacttgtcgctagactggctgacgaaagcggccacgttgtcctcagatggctcccacctcctgaaactcccatgacctctcacattcgctatgaagtggatgtctccgcaggcaacggtgccggaagcgttcagagagtcgagattctcgagggcagaacagagtgtgtgctgtctaacctgcggggcagaaccagatacacatttgctgtgcgcgccaggatggccgaaccttccttcggtggattttggagtgcttggagtgaacccgtgtctctgctgaccccttccgacctcgatcctattccgtggctcggccacctcctcgtgggcctcagcggggcttttggcttcatcatcttagtgtacttgctgatcaactgcaggaacaccgggccatggctgaagaaggtcctgaagtgtaacaccccagacccctcgaagttcttttcccagctgagctcagagcatggaggagacgtccagaagtggctctcttcgcccttcccctcatcgtccttcagccctggcggcctggcacctgagatctcgccactagaagtgctggagagggacaaggtgacgcagctgctcctgcagcaggacaaggtgcctgagcccgcatccttaagcagcaaccactcgctgaccagctgcttcaccaaccagggttacttcttcttccacctcccggatgccttggagatagaggcctgccaggtgttctttactttcgacccctactcagaggaagaccctgatgagggtgtggccggggcacccacagggtcttccccccaacccctgcagcctctgtcaggggaggacgacgcctactgcaccttcccctccagggatgacctgctgctcttctcccccagtctcctcggtggccccagccccccaagcactgcccctgggggcagtggggccggtgaagagaggatgcccccttctttgcaagaaagagtccccagagactgggacccccagcccctggggcctcccaccccaggagtcccagacctggtggattttcagccaccccctgagctggtgctgcgagaggctggggaggaggtccctgacgctggccccagggagggagtcagtttcccctggtccaggcctcctgggcagggggagttcagggcccttaatgctcgcctgcccctgaacactgatgcctacttgtccctccaagaactccagggtcaggacccaactcacttggtgtag

SEQ ID NO: 33 - DNA, 33 bp, synthetic construct
  misc_feature 1..33: note = FFYmut_Rev primer
  source 1..33: mol_type = other DNA
ggggtcgaaagtaaagaacacctggcaggcctc

SEQ ID NO: 34 - DNA, 34 bp, synthetic construct
  misc_feature 1..34: note = FFYmut_Fwd primer
  source 1..34: mol_type = other DNA
tttactttcgacccctactcagaggaagaccctg

SEQ ID NO: 35 - protein, 1228 aa, synthetic construct
  REGION 1..1228: note = ZG-SRG_YFF amino acid sequence
MAQSKHGLTKEMTMKYRMEGCVDGHKFVITGEGIGYPFKGKQAINLCVVEGGPLPFAEDILSAAFMYGNRVFTEYPQDIVDYFKNSCPAGYTWDRSFLFEDGAVCICNADITVSVEENCMYHESKFYGVNFPADGPVMKKMTDNWEPSCEKIIPVPKQGILKGDVSMYLLLKDGGRLRCQFDTVYKAKSVPRKMPDWHFIQHKLTREDRSDAKNQKWHLTEHAIASGSALPRAKRGKPIPNPLLGLDSTSGSGEGRGSLLTCGDVEENPGPDHLGASLWPQVGSLCLLLAGAAWAPPPNLPDPKFESKAALLAARGPEELLCFTERLEDLVCFWEEAASAGVGPGNYSFSYQLEDEPWKLCRLHQAPTARGAVRFWCSLPTADTSSFVPLELRVTAASGAPRYHRVIHINEVVLLDAPVGLVARLADESGHVVLRWLPPPETPMTSHIRYEVDVSAGNGAGSVQRVEILEGRTECVLSNLRGRTRYTFAVRARMAEPSFGGFWSAWSEPVSLLTPSDLDPVVISVGSMGLIISLLCVYFWLERTMPRIPTLKNLEDLVTEYHGNFSAWSGVSKGLAESLQPDYSERLCLVSEIPPKGGALGEGPGASPCNQHSPYWAPPCYTLKPETRRKRGKPIPNPLLGLDSTSGSGATNFSLLKQAGDVEENPGPDHLGASLWPQVGSLCLLLAGAAWAPPPNLPDPKFESKAALLAARGPEELLCFTERLEDLVCFWEEAASAGVGPGNYSFSYQLEDEPWKLCRLHQAPTARGAVRFWCSLPTADTSSFVPLELRVTAASGAPRYHRVIHINEVVLLDAPVGLVARLADESGHVVLRWLPPPETPMTSHIRYEVDVSAGNGAGSVQRVEILEGRTECVLSNLRGRTRYTFAVRARMAEPSFGGFWSAWSEPVSLLTPSDLDPIPWLGHLLVGLSGAFGFIILVYLLINCRNTGPWLKKVLKCNTPDPSKFFSQLSSEHGGDVQKWLSSPFPSSSFSPGGLAPEISPLEVLERDKVTQLLLQQDKVPEPASLSSNHSLTSCFTNQGYFFFHLPDALEIEACQVYFTFDPFSEEDPDEGVAGAPTGSSPQPLQPLSGEDDAYCTFPSRDDLLLFSPSLLGGPSPPSTAPGGSGAGEERMPPSLQERVPRDWDPQPLGPPTPGVPDLVDFQPPPELVLREAGEEVPDAGPREGVSFPWSRPPGQGEFRALNARLPLNTDAYLSLQELQGQDPTHLV

SEQ ID NO: 36 - DNA, 3687 bp, synthetic construct
  misc_feature 1..3687: note = ZG-SRG_YFF nucleic acid sequence
  source 1..3687: mol_type = other DNA
atggcccagtccaagcacggcctgaccaaggagatgaccatgaagtaccgcatggagggctgcgtggacggccacaagttcgtgatcaccggcgagggcatcggctaccccttcaagggcaagcaggccatcaacctgtgcgtggtggagggcggccccttgcccttcgccgaggacatcttgtccgccgccttcatgtacggcaaccgcgtgttcaccgagtacccccaggacatcgtcgactacttcaagaactcctgccccgccggctacacctgggaccgctccttcctgttcgaggacggcgccgtgtgcatctgcaacgccgacatcaccgtgagcgtggaggagaactgcatgtaccacgagtccaagttctacggcgtgaacttccccgccgacggccccgtgatgaagaagatgaccgacaactgggagccctcctgcgagaagatcatccccgtgcccaagcagggcatcttgaagggcgacgtgagcatgtacctgctgctgaaggacggtggccgcttgcgctgccagttcgacaccgtgtacaaggccaagtccgtgccccgcaagatgcccgactggcacttcatccagcacaagctgacccgcgaggaccgcagcgacgccaagaaccagaagtggcacctgaccgagcacgccatcgcctccggctccgccttgcccagggccaagaggggcaagcccattcctaatcctctgctgggcctcgatagcacaagcggcagcggagaaggcagaggctctctgcttacatgcggcgacgtggaagagaaccccggacctgatcacctgggcgcttctctgtggcctcaagtgggatctctgtgtctgctgcttgctggcgctgcttgggctcctcctcctaatctgcccgatcctaagttcgagagcaaggccgctctgctggctgctagaggacctgaggaactgctgtgcttcaccgagagactcgaggacctcgtgtgcttctgggaagaagctgcttctgccggcgttggccctggcaattacagcttcagctaccagctggaagatgagccctggaagctgtgcagactgcatcaggcccctacagctagaggcgctgtgcggttttggtgtagcctgcctacagccgacaccagcagcttcgtgcctctggaactgagagtgacagccgcttctggcgcccctagataccacagagtgatccacatcaacgaggtggtgctgctggatgcccctgttggactggttgccagactggccgatgagtctggacatgtggtgctgagatggctgcctcctccagagacacctatgaccagccacatcagatacgaggtggacgtgtccgccggaaatggcgctggatctgtgcagagagtggaaatcctggaaggccggaccgagtgcgtgctgagcaatctgagaggcagaacccggtacaccttcgccgtcagagccagaatggctgagcctagctttggcggcttttggagcgcttggagcgagccagttagcctgctgacacctagcgatctggaccccgtggttatctctgttggctccatgggattgattatcagccttctctgtgtgtatttctggctggaacggacgatgccccgaattcccaccctgaagaacctagaggatcttgttactgaataccacgggaacttttcggcctggagtggtgtgtctaagggactggctgagagtctgcagccagactacagtgaacgactctgcctcgtcagtgagattcccccaaaaggaggggcccttggggaggggcctggggcctccccatgcaaccagcatagcccctactgggcccccccatgttacaccctaaagcctgaaaccagaagaaagcgcggaaagcctattccaaatccactcctcggcctggacagcacatctggatctggcgccaccaacttcagtctgctgaaacaggccggcgacgtcgaggaaaatcccgggccagatcatctcggagccagtctctggccacaagtcggaagcctgtgtttgttgctggctggtgcagcatgggccccaccaccaaatctccctgatccaaagtttgagtccaaagctgccctgctggccgcaagaggtcccgaagaactcctgtgttttacagagcggcttgaggatctcgtctgtttttgggaagaagccgcctccgctggcgtcggacccggcaattattcctttagctatcagctcgaggacgagccttggaaactgtgtcggctccaccaggctccaactgcaagaggcgccgttagattctggtgctctctgccaaccgccgataccagctcctttgtgcccctcgagcttagagtgactgctgctagcggagccccacggtatcatcgggtcatccatatcaatgaagtcgtcctgctggacgctcccgtgggacttgtcgctagactggctgacgaaagcggccacgttgtcctcagatggctcccacctcctgaaactcccatgacctctcacattcgctatgaagtggatgtctccgcaggcaacggtgccggaagcgttcagagagtcgagattctcgagggcagaacagagtgtgtgctgtctaacctgcggggcagaaccagatacacatttgctgtgcgcgccaggatggccgaaccttccttcggtggattttggagtgcttggagtgaacccgtgtctctgctgaccccttccgacctcgatcctattccgtggctcggccacctcctcgtgggcctcagcggggcttttggcttcatcatcttagtgtacttgctgatcaactgcaggaacaccgggccatggctgaagaaggtcctgaagtgtaacaccccagacccctcgaagttcttttcccagctgagctcagagcatggaggagacgtccagaagtggctctcttcgcccttcccctcatcgtccttcagccctggcggcctggcacctgagatctcgccactagaagtgctggagagggacaaggtgacgcagctgctcctgcagcaggacaaggtgcctgagcccgcatccttaagcagcaaccactcgctgaccagctgcttcaccaaccagggttacttcttcttccacctcccggatgccttggagatagaggcctgccaggtgtactttactttcgaccccttctcagaggaagaccctgatgagggtgtggccggggcacccacagggtcttccccccaacccctgcagcctctgtcaggggaggacgacgcctactgcaccttcccctccagggatgacctgctgctcttctcccccagtctcctcggtggccccagccccccaagcactgcccctgggggcagtggggccggtgaagagaggatgcccccttctttgcaagaaagagtccccagagactgggacccccagcccctggggcctcccaccccaggagtcccagacctggtggattttcagccaccccctgagctggtgctgcgagaggctggggaggaggtccctgacgctggccccagggagggagtcagtttcccctggtccaggcctcctgggcagggggagttcagggcccttaatgctcgcctgcccctgaacactgatgcctacttgtccctccaagaactccagggtcaggacccaactcacttggtgtag

SEQ ID NO: 37 - DNA, 33 bp, synthetic construct
  misc_feature 1..33: note = YFFmut_Rev primer
  source 1..33: mol_type = other DNA
ggggtcgaaagtaaagtacacctggcaggcctc

SEQ ID NO: 38 - DNA, 34 bp, synthetic construct
  misc_feature 1..34: note = YFFmut_Fwd primer
  source 1..34: mol_type = other DNA
tttactttcgaccccttctcagaggaagaccctg

SEQ ID NO: 39 - protein, 1228 aa, synthetic construct
  REGION 1..1228: note = ZG-SRG_FYF amino acid sequence
MAQSKHGLTKEMTMKYRMEGCVDGHKFVITGEGIGYPFKGKQAINLCVVEGGPLPFAEDILSAAFMYGNRVFTEYPQDIVDYFKNSCPAGYTWDRSFLFEDGAVCICNADITVSVEENCMYHESKFYGVNFPADGPVMKKMTDNWEPSCEKIIPVPKQGILKGDVSMYLLLKDGGRLRCQFDTVYKAKSVPRKMPDWHFIQHKLTREDRSDAKNQKWHLTEHAIASGSALPRAKRGKPIPNPLLGLDSTSGSGEGRGSLLTCGDVEENPGPDHLGASLWPQVGSLCLLLAGAAWAPPPNLPDPKFESKAALLAARGPEELLCFTERLEDLVCFWEEAASAGVGPGNYSFSYQLEDEPWKLCRLHQAPTARGAVRFWCSLPTADTSSFVPLELRVTAASGAPRYHRVIHINEVVLLDAPVGLVARLADESGHVVLRWLPPPETPMTSHIRYEVDVSAGNGAGSVQRVEILEGRTECVLSNLRGRTRYTFAVRARMAEPSFGGFWSAWSEPVSLLTPSDLDPVVISVGSMGLIISLLCVYFWLERTMPRIPTLKNLEDLVTEYHGNFSAWSGVSKGLAESLQPDYSERLCLVSEIPPKGGALGEGPGASPCNQHSPYWAPPCYTLKPETRRKRGKPIPNPLLGLDSTSGSGATNFSLLKQAGDVEENPGPDHLGASLWPQVGSLCLLLAGAAWAPPPNLPDPKFESKAALLAARGPEELLCFTERLEDLVCFWEEAASAGVGPGNYSFSYQLEDEPWKLCRLHQAPTARGAVRFWCSLPTADTSSFVPLELRVTAASGAPRYHRVIHINEVVLLDAPVGLVARLADESGHVVLRWLPPPETPMTSHIRYEVDVSAGNGAGSVQRVEILEGRTECVLSNLRGRTRYTFAVRARMAEPSFGGFWSAWSEPVSLLTPSDLDPIPWLGHLLVGLSGAFGFIILVYLLINCRNTGPWLKKVLKCNTPDPSKFFSQLSSEHGGDVQKWLSSPFPSSSFSPGGLAPEISPLEVLERDKVTQLLLQQDKVPEPASLSSNHSLTSCFTNQGYFFFHLPDALEIEACQVFFTYDPFSEEDPDEGVAGAPTGSSPQPLQPLSGEDDAYCTFPSRDDLLLFSPSLLGGPSPPSTAPGGSGAGEERMPPSLQERVPRDWDPQPLGPPTPGVPDLVDFQPPPELVLREAGEEVPDAGPREGVSFPWSRPPGQGEFRALNARLPLNTDAYLSLQELQGQDPTHLV

SEQ ID NO: 40 - DNA, 3687 bp, synthetic construct
  misc_feature 1..3687: note = ZG-SRG_FYF nucleic acid sequence
  source 1..3687: mol_type = other DNA
atggcccagtccaagcacggcctgaccaaggagatgaccatgaagtaccgcatggagggctgcgtggacggccacaagttcgtgatcaccggcgagggcatcggctaccccttcaagggcaagcaggccatcaacctgtgcgtggtggagggcggccccttgcccttcgccgaggacatcttgtccgccgccttcatgtacggcaaccgcgtgttcaccgagtacccccaggacatcgtcgactacttcaagaactcctgccccgccggctacacctgggaccgctccttcctgttcgaggacggcgccgtgtgcatctgcaacgccgacatcaccgtgagcgtggaggagaactgcatgtaccacgagtccaagttctacggcgtgaacttccccgccgacggccccgtgatgaagaagatgaccgacaactgggagccctcctgcgagaagatcatccccgtgcccaagcagggcatcttgaagggcgacgtgagcatgtacctgctgctgaaggacggtggccgcttgcgctgccagttcgacaccgtgtacaaggccaagtccgtgccccgcaagatgcccgactggcacttcatccagcacaagctgacccgcgaggaccgcagcgacgccaagaaccagaagtggcacctgaccgagcacgccatcgcctccggctccgccttgcccagggccaagaggggcaagcccattcctaatcctctgctgggcctcgatagcacaagcggcagcggagaaggcagaggctctctgcttacatgcggcgacgtggaagagaaccccggacctgatcacctgggcgcttctctgtggcctcaagtgggatctctgtgtctgctgcttgctggcgctgcttgggctcctcctcctaatctgcccgatcctaagttcgagagcaaggccgctctgctggctgctagaggacctgaggaactgctgtgcttcaccgagagactcgaggacctcgtgtgcttctgggaagaagctgcttctgccggcgttggccctggcaattacagcttcagctaccagctggaagatgagccctggaagctgtgcagactgcatcaggcccctacagctagaggcgctgtgcggttttggtgtagcctgcctacagccgacaccagcagcttcgtgcctctggaactgagagtgacagccgcttctggcgcccctagataccacagagtgatccacatcaacgaggtggtgctgctggatgcccctgttggactggttgccagactggccgatgagtctggacatgtggtgctgagatggctgcctcctccagagacacctatgaccagccacatcagatacgaggtggacgtgtccgccggaaatggcgctggatctgtgcagagagtggaaatcctggaaggccggaccgagtgcgtgctgagcaatctgagaggcagaacccggtacaccttcgccgtcagagccagaatggctgagcctagctttggcggcttttggagcgcttggagcgagccagttagcctgctgacacctagcgatctggaccccgtggttatctctgttggctccatgggattgattatcagccttctctgtgtgtatttctggctggaacggacgatgccccgaattcccaccctgaagaacctagaggatcttgttactgaataccacgggaacttttcggcctggagtggtgtgtctaagggactggctgagagtctgcagccagactacagtgaacgactctgcctcgtcagtgagattcccccaaaaggaggggcccttggggaggggcctggggcctccccatgcaaccagcatagcccctactgggcccccccatgttacaccctaaagcctgaaaccagaagaaagcgcggaaagcctattccaaatccactcctcggcctggacagcacatctggatctggcgccaccaacttcagtctgctgaaacaggccggcgacgtcgaggaaaatcccgggccagatcatctcggagccagtctctggccacaagtcggaagcctgtgtttgttgctggctggtgcagcatgggccccaccaccaaatctccctgatccaaagtttgagtccaaagctgccctgctggccgcaagaggtcccgaagaactcctgtgttttacagagcggcttgaggatctcgtctgtttttgggaagaagccgcctccgctggcgtcggacccggcaattattcctttagctatcagctcgaggacgagccttggaaactgtgtcggctccaccaggctccaactgcaagaggcgccgttagattctggtgctctctgccaaccgccgataccagctcctttgtgcccctcgagcttagagtgactgctgctagcggagccccacggtatcatcgggtcatccatatcaatgaagtcgtcctgctggacgctcccgtgggacttgtcgctagactggctgacgaaagcggccacgttgtcctcagatggctcccacctcctgaaactcccatgacctctcacattcgctatgaagtggatgtctccgcaggcaacggtgccggaagcgttcagagagtcgagattctcgagggcagaacagagtgtgtgctgtctaacctgcggggcagaaccagatacacatttgctgtgcgcgccaggatggccgaaccttccttcggtggattttggagtgcttggagtgaacccgtgtctctgctgaccccttccgacctcgatcctattccgtggctcggccacctcctcgtgggcctcagcggggcttttggcttcatcatcttagtgtacttgctgatcaactgcaggaacaccgggccatggctgaagaaggtcctgaagtgtaacaccccagacccctcgaagttcttttcccagctgagctcagagcatggaggagacgtccagaagtggctctcttcgcccttcccctcatcgtccttcagccctggcggcctggcacctgagatctcgccactagaagtgctggagagggacaaggtgacgcagctgctcctgcagcaggacaaggtgcctgagcccgcatccttaagcagcaaccactcgctgaccagctgcttcaccaaccagggttacttcttcttccacctcccggatgccttggagatagaggcctgccaggtgttctttacttacgaccccttctcagaggaagaccctgatgagggtgtggccggggcacccacagggtcttccccccaacccctgcagcctctgtcaggggaggacgacgcctactgcaccttcccctccagggatgacctgctgctcttctcccccagtctcctcggtggccccagccccccaagcactgcccctgggggcagtggggccggtgaagagaggatgcccccttctttgcaagaaagagtccccagagactgggacccccagcccctggggcctcccaccccaggagtcccagacctggtggattttcagccaccccctgagctggtgctgcgagaggctggggaggaggtccctgacgctggccccagggagggagtcagtttcccctggtccaggcctcctgggcagggggagttcagggcccttaatgctcgcctgcccctgaacactgatgcctacttgtccctccaagaactccagggtcaggacccaactcacttggtgtag

SEQ ID NO: 41 - DNA, 33 bp, synthetic construct
  misc_feature 1..33: note = FYFmut_Rev primer
  source 1..33: mol_type = other DNA
ggggtcgtaagtaaagaacacctggcaggcctc

SEQ ID NO: 42 - DNA, 34 bp, synthetic construct; identical to SEQ ID NO: 30
  misc_feature 1..34: note = FYFmut_Fwd primer
  source 1..34: mol_type = other DNA

SEQ ID NO: 43 - protein, 1228 aa, synthetic construct
  REGION 1..1228: note = ZG-SRG_FFF amino acid sequence
MAQSKHGLTKEMTMKYRMEGCVDGHKFVITGEGIGYPFKGKQAINLCVVEGGPLPFAEDILSAAFMYGNRVFTEYPQDIVDYFKNSCPAGYTWDRSFLFEDGAVCICNADITVSVEENCMYHESKFYGVNFPADGPVMKKMTDNWEPSCEKIIPVPKQGILKGDVSMYLLLKDGGRLRCQFDTVYKAKSVPRKMPDWHFIQHKLTREDRSDAKNQKWHLTEHAIASGSALPRAKRGKPIPNPLLGLDSTSGSGEGRGSLLTCGDVEENPGPDHLGASLWPQVGSLCLLLAGAAWAPPPNLPDPKFESKAALLAARGPEELLCFTERLEDLVCFWEEAASAGVGPGNYSFSYQLEDEPWKLCRLHQAPTARGAVRFWCSLPTADTSSFVPLELRVTAASGAPRYHRVIHINEVVLLDAPVGLVARLADESGHVVLRWLPPPETPMTSHIRYEVDVSAGNGAGSVQRVEILEGRTECVLSNLRGRTRYTFAVRARMAEPSFGGFWSAWSEPVSLLTPSDLDPVVISVGSMGLIISLLCVYFWLERTMPRIPTLKNLEDLVTEYHGNFSAWSGVSKGLAESLQPDYSERLCLVSEIPPKGGALGEGPGASPCNQHSPYWAPPCYTLKPETRRKRGKPIPNPLLGLDSTSGSGATNFSLLKQAGDVEENPGPDHLGASLWPQVGSLCLLLAGAAWAPPPNLPDPKFESKAALLAARGPEELLCFTERLEDLVCFWEEAASAGVGPGNYSFSYQLEDEPWKLCRLHQAPTARGAVRFWCSLPTADTSSFVPLELRVTAASGAPRYHRVIHINEVVLLDAPVGLVARLADESGHVVLRWLPPPETPMTSHIRYEVDVSAGNGAGSVQRVEILEGRTECVLSNLRGRTRYTFAVRARMAEPSFGGFWSAWSEPVSLLTPSDLDPIPWLGHLLVGLSGAFGFIILVYLLINCRNTGPWLKKVLKCNTPDPSKFFSQLSSEHGGDVQKWLSSPFPSSSFSPGGLAPEISPLEVLERDKVTQLLLQQDKVPEPASLSSNHSLTSCFTNQGYFFFHLPDALEIEACQVFFTFDPFSEEDPDEGVAGAPTGSSPQPLQPLSGEDDAYCTFPSRDDLLLFSPSLLGGPSPPSTAPGGSGAGEERMPPSLQERVPRDWDPQPLGPPTPGVPDLVDFQPPPELVLREAGEEVPDAGPREGVSFPWSRPPGQGEFRALNARLPLNTDAYLSLQELQGQDPTHLV

SEQ ID NO: 44 - DNA, 3687 bp, synthetic construct
  misc_feature 1..3687: note = ZG-SRG_FFF nucleic acid sequence
  source 1..3687: mol_type = other DNA
atggcccagtccaagcacggcctgaccaaggagatgaccatgaagtaccgcatggagggctgcgtggacggccacaagttcgtgatcaccggcgagggcatcggctaccccttcaagggcaagcaggccatcaacctgtgcgtggtggagggcggccccttgcccttcgccgaggacatcttgtccgccgccttcatgtacggcaaccgcgtgttcaccgagtacccccaggacatcgtcgactacttcaagaactcctgccccgccggctacacctgggaccgctccttcctgttcgaggacggcgccgtgtgcatctgcaacgccgacatcaccgtgagcgtggaggagaactgcatgtaccacgagtccaagttctacggcgtgaacttccccgccgacggccccgtgatgaagaagatgaccgacaactgggagccctcctgcgagaagatcatccccgtgcccaagcagggcatcttgaagggcgacgtgagcatgtacctgctgctgaaggacggtggccgcttgcgctgccagttcgacaccgtgtacaaggccaagtccgtgccccgcaagatgcccgactggcacttcatccagcacaagctgacccgcgaggaccgcagcgacgccaagaaccagaagtggcacctgaccgagcacgccatcgcctccggctccgccttgcccagggccaagaggggcaagcccattcctaatcctctgctgggcctcgatagcacaagcggcagcggagaaggcagaggctctctgcttacatgcggcgacgtggaagagaaccccggacctgatcacctgggcgcttctctgtggcctcaagtgggatctctgtgtctgctgcttgctggcgctgcttgggctcctcctcctaatctgcccgatcctaagttcgagagcaaggccgctctgctggctgctagaggacctgaggaactgctgtgcttcaccgagagactcgaggacctcgtgtgcttctgggaagaagctgcttctgccggcgttggccctggcaattacagcttcagctaccagctggaagatgagccctggaagctgtgcagactgcatcaggcccctacagctagaggcgctgtgcggttttggtgtagcctgcctacagccgacaccagcagcttcgtgcctctggaactgagagtgacagccgcttctggcgcccctagataccacagagtgatccacatcaacgaggtggtgctgctggatgcccctgttggactggttgccagactggccgatgagtctggacatgtggtgctgagatggctgcctcctccagagacacctatgaccagccacatcagatacgaggtggacgtgtccgccggaaatggcgctggatctgtgcagagagtggaaatcctggaaggccggaccgagtgcgtgctgagcaatctgagaggcagaacccggtacaccttcgccgtcagagccagaatggctgagcctagctttggcggcttttggagcgcttggagcgagccagttagcctgctgacacctagcgatctggaccccgtggttatctctgttggctccatgggattgattatcagccttctctgtgtgtatttctggctggaacggacgatgccccgaattcccaccctgaagaacctagaggatcttgttactgaataccacgggaacttttcggcctggagtggtgtgtctaagggactggctgagagtctgcagccagactacagtgaacgactctgcctcgtcagtgagattcccccaaaaggaggggcccttggggaggggcctggggcctccccatgcaaccagcatagcccctactgggcccccccatgttacaccctaaagcctgaaaccagaagaaagcgcggaaagcctattccaaatccactcctcggcctggacagcacatctggatctggcgccaccaacttcagtctgctgaaacaggccggcgacgtcgaggaaaatcccgggccagatcatctcggagccagtctctggccacaagtcggaagcctgtgtttgttgctggctggtgcagcatgggccccaccaccaaatctccctgatccaaagtttgagtccaaagctgccctgctggccgcaagaggtcccgaagaactcctgtgttttacagagcggcttgaggatctcgtctgtttttgggaagaagccgcctccgctggcgtcggacccggcaattattcctttagctatcagctcgaggacgagccttggaaactgtgtcggctccaccaggctccaactgcaagaggcgccgttagattctggtgctctctgccaaccgccgataccagctcctttgtgcccctcgagcttagagtgactgctgctagcggagccccacggtatcatcgggtcatccatatcaatgaagtcgtcctgctggacgctcccgtgggacttgtcgctagactggctgacgaaagcggccacgttgtcctcagatggctcccacctcctgaaactcccatgacctctcacattcgctatgaagtggatgtctccgcaggcaacggtgccggaagcgttcagagagtcgagattctcgagggcagaacagagtgtgtgctgtctaacctgcggggcagaaccagatacacatttgctgtgcgcgccaggatggccgaaccttccttcggtggattttggagtgcttggagtgaacccgtgtctctgctgaccccttccgacctcgatcctattccgtggctcggccacctcctcgtgggcctcagcggggcttttggcttcatcatcttagtgtacttgctgatcaactgcaggaacaccgggccatggctgaagaaggtcctgaagtgtaacaccccagacccctcgaagttcttttcccagctgagctcagagcatggaggagacgtccagaagtggctctcttcgcccttcccctcatcgtccttcagccctggcggcctggcacctgagatctcgccactagaagtgctggagagggacaaggtgacgcagctgctcctgcagcaggacaaggtgcctgagcccgcatccttaagcagcaaccactcgctgaccagctgcttcaccaaccagggttacttcttcttccacctcccggatgccttggagatagaggcctgccaggtgttctttactttcgaccccttctcagaggaagaccctgatgagggtgtggccggggcacccacagggtcttccccccaacccctgcagcctctgtcaggggaggacgacgcctactgcaccttcccctccagggatgacctgctgctcttctcccccagtctcctcggtggccccagccccccaagcactgcccctgggggcagtggggccggtgaagagaggatgcccccttctttgcaagaaagagtccccagagactgggacccccagcccctggggcctcccaccccaggagtcccagacctggtggattttcagccaccccctgagctggtgctgcgagaggctggggaggaggtccctgacgctggccccagggagggagtcagtttcccctggtccaggcctcctgggcagggggagttcagggcccttaatgctcgcctgcccctgaacactgatgcctacttgtccctccaagaactccagggtcaggacccaactcacttggtgtag

SEQ ID NO: 45 - DNA, 33 bp, synthetic construct; identical to SEQ ID NO: 33
  misc_feature 1..33: note = FFFmut_Rev primer
  source 1..33: mol_type = other DNA

SEQ ID NO: 46 - DNA, 34 bp, synthetic construct; identical to SEQ ID NO: 38
  misc_feature 1..34: note = FFFmut_Fwd primer
  source 1..34: mol_type = other DNA

SEQ ID NO: 47 - protein, 958 aa, synthetic construct
  REGION 1..958: note = SRG_YYY amino acid sequence
MDHLGASLWPQVGSLCLLLAGAAWAPPPNLPDPKFESKAALLAARGPEELLCFTERLEDLVCFWEEAASAGVGPGNYSFSYQLEDEPWKLCRLHQAPTARGAVRFWCSLPTADTSSFVPLELRVTAASGAPRYHRVIHINEVVLLDAPVGLVARLADESGHVVLRWLPPPETPMTSHIRYEVDVSAGNGAGSVQRVEILEGRTECVLSNLRGRTRYTFAVRARMAEPSFGGFWSAWSEPVSLLTPSDLDPVVISVGSMGLIISLLCVYFWLERTMPRIPTLKNLEDLVTEYHGNFSAWSGVSKGLAESLQPDYSERLCLVSEIPPKGGALGEGPGASPCNQHSPYWAPPCYTLKPETRRKRGKPIPNPLLGLDSTSGSGATNFSLLKQAGDVEENPGPDHLGASLWPQVGSLCLLLAGAAWAPPPNLPDPKFESKAALLAARGPEELLCFTERLEDLVCFWEEAASAGVGPGNYSFSYQLEDEPWKLCRLHQAPTARGAVRFWCSLPTADTSSFVPLELRVTAASGAPRYHRVIHINEVVLLDAPVGLVARLADESGHVVLRWLPPPETPMTSHIRYEVDVSAGNGAGSVQRVEILEGRTECVLSNLRGRTRYTFAVRARMAEPSFGGFWSAWSEPVSLLTPSDLDPIPWLGHLLVGLSGAFGFIILVYLLINCRNTGPWLKKVLKCNTPDPSKFFSQLSSEHGGDVQKWLSSPFPSSSFSPGGLAPEISPLEVLERDKVTQLLLQQDKVPEPASLSSNHSLTSCFTNQGYFFFHLPDALEIEACQVYFTYDPYSEEDPDEGVAGAPTGSSPQPLQPLSGEDDAYCTFPSRDDLLLFSPSLLGGPSPPSTAPGGSGAGEERMPPSLQERVPRDWDPQPLGPPTPGVPDLVDFQPPPELVLREAGEEVPDAGPREGVSFPWSRPPGQGEFRALNARLPLNTDAYLSLQELQGQDPTHLV

SEQ ID NO: 48 - DNA, 2877 bp, synthetic construct
  misc_feature 1..2877: note = SRG_YYY nucleic acid sequence
  source 1..2877: mol_type = other DNA
atggatcacctgggcgcttctctgtggcctcaagtgggatctctgtgtctgctgcttgctggcgctgcttgggctcctcctcctaatctgcccgatcctaagttcgagagcaaggccgctctgctggctgctagaggacctgaggaactgctgtgcttcaccgagagactcgaggacctcgtgtgcttctgggaagaagctgcttctgccggcgttggccctggcaattacagcttcagctaccagctggaagatgagccctggaagctgtgcagactgcatcaggcccctacagctagaggcgctgtgcggttttggtgtagcctgcctacagccgacaccagcagcttcgtgcctctggaactgagagtgacagccgcttctggcgcccctagataccacagagtgatccacatcaacgaggtggtgctgctggatgcccctgttggactggttgccagactggccgatgagtctggacatgtggtgctgagatggctgcctcctccagagacacctatgaccagccacatcagatacgaggtggacgtgtccgccggaaatggcgctggatctgtgcagagagtggaaatcctggaaggccggaccgagtgcgtgctgagcaatctgagaggcagaacccggtacaccttcgccgtcagagccagaatggctgagcctagctttggcggcttttggagcgcttggagcgagccagttagcctgctgacacctagcgatctggaccccgtggttatctctgttggctccatgggattgattatcagccttctctgtgtgtatttctggctggaacggacgatgccccgaattcccaccctgaagaacctagaggatcttgttactgaataccacgggaacttttcggcctggagtggtgtgtctaagggactggctgagagtctgcagccagactacagtgaacgactctgcctcgtcagtgagattcccccaaaaggaggggcccttggggaggggcctggggcctccccatgcaaccagcatagcccctactgggcccccccatgttacaccctaaagcctgaaaccagaagaaagcgcggaaagcctattccaaatccactcctcggcctggacagcacatctggatctggcgccaccaacttcagtctgctgaaacaggccggcgacgtcgaggaaaatcccgggccagatcatctcggagccagtctctggccacaagtcggaagcctgtgtttgttgctggctggtgcagcatgggccccaccaccaaatctccctgatccaaagtttgagtccaaagctgccctgctggccgcaagaggtcccgaagaactcctgtgttttacagagcggcttgaggatctcgtctgtttttgggaagaagccgcctccgctggcgtcggacccggcaattattcctttagctatcagctcgaggacgagccttggaaactgtgtcggctccaccaggctccaactgcaagaggcgccgttagattctggtgctctctgccaaccgccgataccagctcctttgtgcccctcgagcttagagtgactgctgctagcggagccccacggtatcatcgggtcatccatatcaatgaagtcgtcctgctggacgctcccgtgggacttgtcgctagactggctgacgaaagcggccacgttgtcctcagatggctcccacctcctgaaactcccatgacctctcacattcgctatgaagtggatgtctccgcaggcaacggtgccggaagcgttcagagagtcgagattctcgagggcagaacagagtgtgtgctgtctaacctgcggggcagaaccagatacacatttgctgtgcgcgccaggatggccgaaccttccttcggtggattttggagtgcttggagtgaacccgtgtctctgctgaccccttccgacctcgatcctattccgtggctcggccacctcctcgtgggcctcagcggggcttttggcttcatcatcttagtgtacttgctgatcaactgcaggaacaccgggccatggctgaagaaggtcctgaagtgtaacaccccagacccctcgaagttcttttcccagctgagctcagagcatggaggagacgtccagaagtggctctcttcgcccttcccctcatcgtccttcagccctggcggcctggcacctgagatctcgccactagaagtgctggagagggacaaggtgacgcagctgctcctgcagcaggacaaggtgcctgagcccgcatccttaagcagcaaccactcgctgaccagctgcttcaccaaccagggttacttcttcttccacctcccggatgccttggagatagaggcctgccaggtgtactttacttacgacccctactcagaggaagaccctgatgagggtgtggccggggcacccacagggtcttccccccaacccctgcagcctctgtcaggggaggacgacgcctactgcaccttcccctccagggatgacctgctgctcttctcccccagtctcctcggtggccccagccccccaagcactgcccctgggggcagtggggccggtgaagagaggatgcccccttctttgcaagaaagagtccccagagactgggacccccagcccctggggcctcccaccccaggagtcccagacctggtggattttcagccaccccctgagctggtgctgcgagaggctggggaggaggtccctgacgctggccccagggagggagtcagtttcccctggtccaggcctcctgggcagggggagttcagggcccttaatgctcgcctgcccctgaacactgatgcctacttgtccctccaagaactccagggtcaggacccaactcacttggtgtag

SEQ ID NO: 49 - DNA, 57 bp, synthetic construct
  misc_feature 1..57: note = SRG_M5InfFwd primer
  source 1..57: mol_type = other DNA
gagctcggatctcacgtgccaccatggatcacctgggcgcttctctgtggcctcaag

SEQ ID NO: 50 - protein, 958 aa, synthetic construct
  REGION 1..958: note = SRG_FFF amino acid sequence
MDHLGASLWPQVGSLCLLLAGAAWAPPPNLPDPKFESKAALLAARGPEELLCFTERLEDLVCFWEEAASAGVGPGNYSFSYQLEDEPWKLCRLHQAPTARGAVRFWCSLPTADTSSFVPLELRVTAASGAPRYHRVIHINEVVLLDAPVGLVARLADESGHVVLRWLPPPETPMTSHIRYEVDVSAGNGAGSVQRVEILEGRTECVLSNLRGRTRYTFAVRARMAEPSFGGFWSAWSEPVSLLTPSDLDPVVISVGSMGLIISLLCVYFWLERTMPRIPTLKNLEDLVTEYHGNFSAWSGVSKGLAESLQPDYSERLCLVSEIPPKGGALGEGPGASPCNQHSPYWAPPCYTLKPETRRKRGKPIPNPLLGLDSTSGSGATNFSLLKQAGDVEENPGPDHLGASLWPQVGSLCLLLAGAAWAPPPNLPDPKFESKAALLAARGPEELLCFTERLEDLVCFWEEAASAGVGPGNYSFSYQLEDEPWKLCRLHQAPTARGAVRFWCSLPTADTSSFVPLELRVTAASGAPRYHRVIHINEVVLLDAPVGLVARLADESGHVVLRWLPPPETPMTSHIRYEVDVSAGNGAGSVQRVEILEGRTECVLSNLRGRTRYTFAVRARMAEPSFGGFWSAWSEPVSLLTPSDLDPIPWLGHLLVGLSGAFGFIILVYLLINCRNTGPWLKKVLKCNTPDPSKFFSQLSSEHGGDVQKWLSSPFPSSSFSPGGLAPEISPLEVLERDKVTQLLLQQDKVPEPASLSSNHSLTSCFTNQGYFFFHLPDALEIEACQVFFTFDPFSEEDPDEGVAGAPTGSSPQPLQPLSGEDDAYCTFPSRDDLLLFSPSLLGGPSPPSTAPGGSGAGEERMPPSLQERVPRDWDPQPLGPPTPGVPDLVDFQPPPELVLREAGEEVPDAGPREGVSFPWSRPPGQGEFRALNARLPLNTDAYLSLQELQGQDPTHLV

SEQ ID NO: 51 - DNA, 2877 bp, synthetic construct
  misc_feature 1..2877: note = SRG_FFF nucleic acid sequence
  source 1..2877: mol_type = other DNA
atggatcacctgggcgcttctctgtggcctcaagtgggatctctgtgtctgctgcttgctggcgctgcttgggctcctcctcctaatctgcccgatcctaagttcgagagcaaggccgctctgctggctgctagaggacctgaggaactgctgtgcttcaccgagagactcgaggacctcgtgtgcttctgggaagaagctgcttctgccggcgttggccctggcaattacagcttcagctaccagctggaagatgagccctggaagctgtgcagactgcatcaggcccctacagctagaggcgctgtgcggttttggtgtagcctgcctacagccgacaccagcagcttcgtgcctctggaactgagagtgacagccgcttctggcgcccctagataccacagagtgatccacatcaacgaggtggtgctgctggatgcccctgttggactggttgccagactggccgatgagtctggacatgtggtgctgagatggctgcctcctccagagacacctatgaccagccacatcagatacgaggtggacgtgtccgccggaaatggcgctggatctgtgcagagagtggaaatcctggaaggccggaccgagtgcgtgctgagcaatctgagaggcagaacccggtacaccttcgccgtcagagccagaatggctgagcctagctttggcggcttttggagcgcttggagcgagccagttagcctgctgacacctagcgatctggaccccgtggttatctctgttggctccatgggattgattatcagccttctctgtgtgtatttctggctggaacggacgatgccccgaattcccaccctgaagaacctagaggatcttgttactgaataccacgggaacttttcggcctggagtggtgtgtctaagggactggctgagagtctgcagccagactacagtgaacgactctgcctcgtcagtgagattcccccaaaaggaggggcccttggggaggggcctggggcctccccatgcaaccagcatagcccctactgggcccccccatgttacaccctaaagcctgaaaccagaagaaagcgcggaaagcctattccaaatccactcctcggcctggacagcacatctggatctggcgccaccaacttcagtctgctgaaacaggccggcgacgtcgaggaaaatcccgggccagatcatctcggagccagtctctggccacaagtcggaagcctgtgtttgttgctggctggtgcagcatgggccccaccaccaaatctccctgatccaaagtttgagtccaaagctgccctgctggccgcaagaggtcccgaagaactcctgtgttttacagagcggcttgaggatctcgtctgtttttgggaagaagccgcctccgctggcgtcggacccggcaattattcctttagctatcagctcgaggacgagccttggaaactgtgtcggctccaccaggctccaactgcaagaggcgccgttagattctggtgctctctgccaaccgccgataccagctcctttgtgcccctcgagcttagagtgactgctgctagcggagccccacggtatcatcgggtcatccatatcaatgaagtcgtcctgctggacgctcccgtgggacttgtcgctagactggctgacgaaagcggccacgttgtcctcagatggctcccacctcctgaaactcccatgacctctcacattcgctatgaagtggatgtctccgcaggcaacggtgccggaagcgttcagagagtcgagattctcgagggcagaacagagtgtgtgctgtctaacctgcggggcagaaccagatacacatttgctgtgcgcgccaggatggccgaaccttccttcggtggattttggagtgcttggagtgaacccgtgtctctgctgaccccttccgacctcgatcctattccgtggctcggccacctcctcgtgggcctcagcggggcttttggcttcatcatcttagtgtacttgctgatcaactgcaggaacaccgggccatggctgaagaaggtcctgaagtgtaacaccccagacccctcgaagttcttttcccagctgagctcagagcatggaggagacgtccagaagtggctctcttcgcccttcccctcatcgtccttcagccctggcggcctggcacctgagatctcgccactagaagtgctggagagggacaaggtgacgcagctgctcctgcagcaggacaaggtgcctgagcccgcatccttaagcagcaaccactcgctgaccagctgcttcaccaaccagggttacttcttcttccacctcccggatgccttggagatagaggcctgccaggtgttctttactttcgaccccttctcagaggaagaccctgatgagggtgtggccggggcacccacagggtcttccccccaacccctgcagcctctgtcaggggaggacgacgcctactgcaccttcccctccagggatgacctgctgctcttctcccccagtctcctcggtggccccagccccccaagcactgcccctgggggcagtggggccggtgaagagaggatgcccccttctttgcaagaaagagtccccagagactgggacccccagcccctggggcctcccaccccaggagtcccagacctggtggattttcagccaccccctgagctggtgctgcgagaggctggggaggaggtccctgacgctggccccagggagggagtcagtttcccctggtccaggcctcctgggcagggggagttcagggcccttaatgctcgcctgcccctgaacactgatgcctacttgtccctccaagaactccagggtcaggacccaactcacttggtgtag

SEQ ID NO: 52 - protein, 1524 aa, synthetic construct
  REGION 1..1524: note = EL-SRG_FFF amino acid sequence
MEREKNVVYGPEPKHPLGNFTAGEMLYNALHKHSHIPQAILDVMGNESLSYQEFFDTTVKLGQSLQNCGYKMNDVVSICAENNKRFFIPIISAWYIGMVVAPVNEDYIPDELCKVTGISKPILVFTTRKILPKVLEVKDRTNYIKRIIILDSEENLLGCESLHNFMSRYSDNNLQTFKPLHYDPVDQVAAILCSSGTTGLPKGVMQTHRNICVRLTHASDPRVGTQLIPGVSVLAYLPFFHAFGFSINLGYFMVGLRVVMLRRFNQEVFLKAIQDYEVRSVINVPSTILFLSKSPLVDKYDLSTLAELCCGAAPLAKEVAEIAVKRLNLPGIRCGYGLTESTSANIHTLHNEFKSGSLGKVTPYMAAKIIDRNTGEALGPNQVGELCIWGPMVTKGYVNNPQATKEAIDDDGWLHSGDFGYYDEDEYFYIVDRYKELIKYKGYQVAPVELEEILLQHPGIRDVAVVGIPDIEAGELPAGFVVKQPGAQLTAKEVYDFLAQRVSHSKYLRGGVRFVDSIPRNVTGKISRKELREALMEKASKLRAKRGSGEGRGSLLTCGDVEENPGPDHLGASLWPQVGSLCLLLAGAAWAPPPNLPDPKFESKAALLAARGPEELLCFTERLEDLVCFWEEAASAGVGPGNYSFSYQLEDEPWKLCRLHQAPTARGAVRFWCSLPTADTSSFVPLELRVTAASGAPRYHRVIHINEVVLLDAPVGLVARLADESGHVVLRWLPPPETPMTSHIRYEVDVSAGNGAGSVQRVEILEGRTECVLSNLRGRTRYTFAVRARMAEPSFGGFWSAWSEPVSLLTPSDLDPVVISVGSMGLIISLLCVYFWLERTMPRIPTLKNLEDLVTEYHGNFSAWSGVSKGLAESLQPDYSERLCLVSEIPPKGGALGEGPGASPCNQHSPYWAPPCYTLKPETRRKRGKPIPNPLLGLDSTSGSGATNFSLLKQAGDVEENPGPDHLGASLWPQVGSLCLLLAGAAWAPPPNLPDPKFESKAALLAARGPEELLCFTERLEDLVCFWEEAASAGVGPGNYSFSYQLEDEPWKLCRLHQAPTARGAVRFWCSLPTADTSSFVPLELRVTAASGAPRYHRVIHINEVVLLDAPVGLVARLADESGHVVLRWLPPPETPMTSHIRYEVDVSAGNGAGSVQRVEILEGRTECVLSNLRGRTRYTFAVRARMAEPSFGGFWSAWSEPVSLLTPSDLDPIPWLGHLLVGLSGAFGFIILVYLLINCRNTGPWLKKVLKCNTPDPSKFFSQLSSEHGGDVQKWLSSPFPSSSFSPGGLAPEISPLEVLERDKVTQLLLQQDKVPEPASLSSNHSLTSCFTNQGYFFFHLPDALEIEACQVFFTFDPFSEEDPDEGVAGAPTGSSPQPLQPLSGEDDAYCTFPSRDDLLLFSPSLLGGPSPPSTAPGGSGAGEERMPPSLQERVPRDWDPQPLGPPTPGVPDLVDFQPPPELVLREAGEEVPDAGPREGVSFPWSRPPGQGEFRALNARLPLNTDAYLSLQELQGQDPTHLV

SEQ ID NO: 53 - DNA, 4650 bp, synthetic construct
  misc_feature 1..4650: note = EL-SRG_FFF nucleic acid sequence
  source 1..4650: mol_type = other DNA
atggagagagagaagaacgtggtgtacggccccgagcccaagcaccctctgggcaacttcaccgccggcgagatgctgtacaacgctctgcacaagcactcccacatcccccaggccatcctggacgtgatgggcaacgagtccctttcctaccaggagttcttcgacactactgtgaagctgggccagagcctccagaactgtggctacaagatgaacgatgtcgtgtcgatctgtgcagagaacaacaagagattcttcatccccatcatctccgcctggtacatcggcatggtggtggcccctgtgaacgaggactatatcccagacgagctgtgtaaagtgaccggcatctccaagccgatcctggtcttcaccactaggaagatcctgcctaaggttttggaggttaaagacagaaccaactacataaagaggatcatcatactggactctgaagagaacctgctgggctgcgagagcctgcacaacttcatgtccaggtactccgacaacaacctccaaacattcaagcctctgcactacgaccctgtggaccaggtagccgccatcctgtgctcctccggcacaaccggcctgcctaaaggcgtgatgcagacccacaggaacatctgtgtgagactcacacacgcatctgaccccagagtgggtacacaactcatccccggcgtatccgtgctggcctacctgccattcttccacgccttcggcttcagtatcaacctgggctatttcatggtgggcctgagagtggtgatgctccgaaggtttaaccaggaggtgttcctgaaggccatccaggactacgaggtgaggagcgtgatcaacgttccctccacaatcctgttcctgtccaagagccctctggtggacaagtacgacctatccaccctggcggagctgtgctgtggagccgctcctctggcgaaggaggtggccgagatcgccgtgaagaggctgaacctgccagggatacggtgtggctacggtctaacagagtctacctccgccaacatccatactctgcacaacgagttcaagtccggctccctgggcaaggtgacaccttacatggccgccaagatcatcgacaggaacaccggcgaggccctgggtccaaaccaggtgggcgagctgtgcatctggggacctatggtaacaaaaggctatgtgaacaacccacaggctactaaggaggccatcgacgacgacggctggctgcactctggcgacttcggctactacgacgaggacgagtatttctacatcgtggaccggtacaaggagctgatcaaatacaagggctatcaggtcgcccctgtggagctggaggagatcctccttcagcacccaggcatcagggacgtggccgtcgtgggtatccctgacatcgaggccggcgagctgccagccggcttcgtggtgaagcagcccggcgcccaactcaccgctaaggaggtgtacgacttcctggcccagagggtgtctcactccaagtacctgaggggcggcgtaaggttcgtggactctatccccaggaacgtgacaggcaagattagtcgaaaagagctgagggaggccctgatggagaaggcttctaagctgagagccaagagaggcagcggcgaaggcagaggatctctgctgacatgtggcgacgtggaagagaatcccggacctgatcacctgggcgcttctctgtggcctcaagtgggatctctgtgtctgctgcttgctggcgctgcttgggctcctcctcctaatctgcccgatcctaagttcgagagcaaggccgctctgctggctgctagaggacctgaggaactgctgtgcttcaccgagagactcgaggacctcgtgtgcttctgggaagaagctgcttctgccggcgttggccctggcaattacagcttcagctaccagctggaagatgagccctggaagctgtgcagactgcatcaggcccctacagctagaggcgctgtgcggttttggtgtagcctgcctacagccgacaccagcagcttcgtgcctctggaactgagagtgacagccgcttctggcgcccctagataccacagagtgatccacatcaacgaggtggtgctgctggatgcccctgttggactggttgccagactggccgatgagtctggacatgtggtgctgagatggctgcctcctccagagacacctatgaccagccacatcagatacgaggtggacgtgtccgccggaaatggcgctggatctgtgcagagagtggaaatcctggaaggccggaccgagtgcgtgctgagcaatctgagaggcagaacccggtacaccttcgccgtcagagccagaatggctgagcctagctttggcggcttttggagcgcttggagcgagccagttagcctgctgacacctagcgatctggaccccgtggttatctctgttggctccatgggattgattatcagccttctctgtgtgtatttctggctggaacggacgatgccccgaattcccaccctgaagaacctagaggatcttgttactgaataccacgggaacttttcggcctggagtggtgtgtctaagggactggctgagagtctgcagccagactacagtgaacgactctgcctcgtcagtgagattcccccaaaaggaggggcccttggggaggggcctggggcctccccatgcaaccagcatagcccctactgggcccccccatgttacaccctaaagcctgaaaccagaagaaagcgcggaaagcctattccaaatccactcctcggcctggacagcacatctggatctggcgccaccaacttcagtctgctgaaacaggccggcgacgtcgaggaaaatcccgggccagatcatctcggagccagtctctggccacaagtcggaagcctgtgtttgttgctggctggtgcagcatgggccccaccaccaaatctccctgatccaaagtttgagtccaaagctgccctgctggccgcaagaggtcccgaagaactcctgtgttttacagagcggcttgaggatctcgtctgtttttgggaagaagccgcctccgctggcgtcggacccggcaattattcctttagctatcagctcgaggacgagccttggaaactgtgtcggctccaccaggctccaactgcaagaggcgccgttagattctggtgctctctgccaaccgccgataccagctcctttgtgcccctcgagcttagagtgactgctgctagcggagccccacggtatcatcgggtcatccatatcaatgaagtcgtcctgctggacgctcccgtgggacttgtcgctagactggctgacgaaagcggccacgttgtcctcagatggctcccacctcctgaaactcccatgacctctcacattcgctatgaagtggatgtctccgcaggcaacggtgccggaagcgttcagagagtcgagattctcgagggcagaacagagtgtgtgctgtctaacctgcggggcagaaccagatacacatttgctgtgcgcgccaggatggccgaaccttccttcggtggattttggagtgcttggagtgaacccgtgtctctgctgaccccttccgacctcgatcctattccgtggctcggccacctcctcgtgggcctcagcggggcttttggcttcatcatcttagtgtacttgctgatcattccgtggctcggccacctcctcgtgggcctcagcggggcttttggcttcatcatcttagtgtacttgctgatcaactgcaggaacaccgggccatggctgaagaaggtcctgaagtgtaacaccccagacccctcgaagttcttttcccagctgagctcagagcatggaggagacgtccagaagtggctctcttcgcccttcccctcatcgtccttcagccctggcggcctggcacctgagatctcgccactagaagtgctggagagggacaaggtgacgcagctgctcctgcagcaggacaaggtgcctgagcccgcatccttaagcagcaaccactcgctgaccagctgcttcaccaaccagggttacttcttcttccacctcccggatgccttggagatagaggcctgccaggtgttctttactttcgaccccttctcagaggaagaccctgatgagggtgtggccggggcacccacagggtcttccccccaacccctgcagcctctgtcaggggaggacgacgcctactgcaccttcccctccagggatgacctgctgctcttctcccccagtctcctcggtggccccagccccccaagcactgcccctgggggcagtggggccggtgaagagaggatgcccccttctttgcaagaaagagtccccagagactgggacccccagcccctggggcctcccaccccaggagtcccagacctggtggattttcagccaccccctgagctggtgctgcgagaggctggggaggaggtccctgacgctggccccagggagggagtcagtttcccctggtccaggcctcctgggcagggggagttcagggcccttaatgctcgcctgcccctgaacactgatgcctacttgtccctccaagaactccagggtcaggacccaactcacttggtgtag

SEQ ID NO: 54 - DNA, 47 bp, synthetic construct
  misc_feature 1..47: note = ELSRG-EL_M5InfFwd primer
  source 1..47: mol_type = other DNA
gagctcggatctcacgtgccaccatggagagagagaagaacgtggtg

SEQ ID NO: 55 - DNA, 67 bp, synthetic construct
  misc_feature 1..67: note = ELSRG-EL_M5InfRev primer
  source 1..67: mol_type = other DNA
tgtcagcagagatcctctgccttcgccgctgcctctcttggctctcagcttagaagccttctccatc

SEQ ID NO: 56 - DNA, 66 bp, synthetic construct
  misc_feature 1..66: note = ELSRG-SRG_M5InfFwd primer
  source 1..66: mol_type = other DNA
ggatctctgctgacatgtggcgacgtggaagagaatcccggacctgatcacctgggcgcttctctg

SEQ ID NO: 57 - protein, 489 aa, synthetic construct
  REGION 1..489: note = FMC28z amino acid sequence
MLLLVTSLLLCELPHPAFLLIPDIQMTQTTSSLSASLGDRVTISCRASQDISKYLNWYQQKPDGTVKLLIYHTSRLHSGVPSRFSGSGSGTDYSLTISNLEQEDIATYFCQQGNTLPYTFGGGTKLEITGSTSGSGKPGSGEGSTKGEVKLQESGPGLVAPSQSLSVTCTVSGVSLPDYGVSWIRQPPRKGLEWLGVIWGSETTYYNSALKSRLTIIKDNSKSQVFLKMNSLQTDDTAIYYCAKHYYYGGSYAMDYWGQGTSVTVSSAAAIEVMYPPPYLDNEKSNGTIIHVKGKHLCPSPLFPGPSKPFWVLVVVGGVLACYSLLVTVAFIIFWVRSKRSRLLHSDYMNMTPRRPGPTRKHYQPYAPPRDFAAYRSRVKFSRSADAPAYQQGQNQLYNELNLGRREEYDVLDKRRGRDPEMGGKPRRKNPQEGLYNELQKDKMAEAYSEIGMKGERRRGKGHDGLYQGLSTATKDTYDALHMQALPPR

SEQ ID NO: 58 - DNA, 1470 bp, synthetic construct
  misc_feature 1..1470: note = FMC28z nucleic acid sequence
  source 1..1470: mol_type = other DNA
atgctgctgctggtcacatctctgctgctgtgcgagctgccccatcctgcctttctgctgatccccgacatccagatgacccagaccacaagcagcctgtctgccagcctgggcgatagagtgaccatcagctgtagagccagccaggacatcagcaagtacctgaactggtatcagcaaaagcccgacggcaccgtgaagctgctgatctaccacaccagcagactgcacagcggcgtgccaagcagattttctggcagcggctctggcaccgactacagcctgaccatctccaacctggaacaagaggacattgccacctacttttgccagcaaggcaacaccctgccttacacctttggcggaggcaccaagctggaaatcaccggctctacaagcggcagcggcaaacctggatctggcgagggatctaccaagggcgaagtgaaactgcaagagtctggccctggactggtggccccatctcagtctctgagcgtgacctgtacagtcagcggagtgtccctgcctgattacggcgtgtcctggatcagacagcctcctcggaaaggcctggaatggctgggagtgatctggggcagcgagacaacctactacaacagcgccctgaagtcccggctgaccatcatcaaggacaactccaagagccaggtgttcctgaagatgaacagcctgcagaccgacgacaccgccatctactattgcgccaagcactactactacggcggcagctacgctatggactattggggccagggcaccagcgtgacagtttcttctgccgccgctatcgaagtgatgtaccctccaccttacctggacaacgagaagtccaacggcaccatcatccatgtgaagggcaaacatctgtgcccctctccactgttccccggacctagcaagcctttctgggtgctcgttgttgttggcggcgtgctggcctgttatagcctgctggttaccgtggccttcatcatcttttgggtccgaagcaagagaagccggctgctgcacagcgactacatgaacatgacccctagacggcccggaccaaccagaaagcactaccagccttacgctcctcctagagacttcgccgcctaccggtccagagtgaagttcagcagatccgccgatgctcccgcctatcagcagggccagaaccagctgtacaacgagctgaacctggggagaagagaagagtacgacgtgctggacaagcggagaggacgcgatcctgaaatgggcggcaagcctcggagaaagaatccccaagagggactgtataatgagctgcagaaagacaagatggccgaggcctacagcgagatcggcatgaagggcgagcgcagaagaggcaaaggacacgatggcctgtatcagggcctgagcaccgccactaaggacacctacgatgcactgcacatgcaggccctgcctccaagataa

SEQ ID NO: 59 - protein, 1471 aa, synthetic construct
  REGION 1..1471: note = FMC28z-SRG_FFF amino acid sequence
MLLLVTSLLLCELPHPAFLLIPDIQMTQTTSSLSASLGDRVTISCRASQDISKYLNWYQQKPDGTVKLLIYHTSRLHSGVPSRFSGSGSGTDYSLTISNLEQEDIATYFCQQGNTLPYTFGGGTKLEITGSTSGSGKPGSGEGSTKGEVKLQESGPGLVAPSQSLSVTCTVSGVSLPDYGVSWIRQPPRKGLEWLGVIWGSETTYYNSALKSRLTIIKDNSKSQVFLKMNSLQTDDTAIYYCAKHYYYGGSYAMDYWGQGTSVTVSSAAAIEVMYPPPYLDNEKSNGTIIHVKGKHLCPSPLFPGPSKPFWVLVVVGGVLACYSLLVTVAFIIFWVRSKRSRLLHSDYMNMTPRRPGPTRKHYQPYAPPRDFAAYRSRVKFSRSADAPAYQQGQNQLYNELNLGRREEYDVLDKRRGRDPEMGGKPRRKNPQEGLYNELQKDKMAEAYSEIGMKGERRRGKGHDGLYQGLSTATKDTYDALHMQALPPRRAKRGSGEGRGSLLTCGDVEENPGPDHLGASLWPQVGSLCLLLAGAAWAPPPNLPDPKFESKAALLAARGPEELLCFTERLEDLVCFWEEAASAGVGPGNYSFSYQLEDEPWKLCRLHQAPTARGAVRFWCSLPTADTSSFVPLELRVTAASGAPRYHRVIHINEVVLLDAPVGLVARLADESGHVVLRWLPPPETPMTSHIRYEVDVSAGNGAGSVQRVEILEGRTECVLSNLRGRTRYTFAVRARMAEPSFGGFWSAWSEPVSLLTPSDLDPVVISVGSMGLIISLLCVYFWLERTMPRIPTLKNLEDLVTEYHGNFSAWSGVSKGLAESLQPDYSERLCLVSEIPPKGGALGEGPGASPCNQHSPYWAPPCYTLKPETRRKRGKPIPNPLLGLDSTSGSGATNFSLLKQAGDVEENPGPDHLGASLWPQVGSLCLLLAGAAWAPPPNLPDPKFESKAALLAARGPEELLCFTERLEDLVCFWEEAASAGVGPGNYSFSYQLEDEPWKLCRLHQAPTARGAVRFWCSLPTADTSSFVPLELRVTAASGAPRYHRVIHINEVVLLDAPVGLVARLADESGHVVLRWLPPPETPMTSHIRYEVDVSAGNGAGSVQRVEILEGRTECVLSNLRGRTRYTFAVRARMAEPSFGGFWSAWSEPVSLLTPSDLDPIPWLGHLLVGLSGAFGFIILVYLLINCRNTGPWLKKVLKCNTPDPSKFFSQLSSEHGGDVQKWLSSPFPSSSFSPGGLAPEISPLEVLERDKVTQLLLQQDKVPEPASLSSNHSLTSCFTNQGYFFFHLPDALEIEACQVFFTFDPFSEEDPDEGVAGAPTGSSPQPLQPLSGEDDAYCTFPSRDDLLLFSPSLLGGPSPPSTAPGGSGAGEERMPPSLQERVPRDWDPQPLGPPTPGVPDLVDFQPPPELVLREAGEEVPDAGPREGVSFPWSRPPGQGEFRALNARLPLNTDAYLSLQELQGQDPTHLV

SEQ ID NO: 60 - DNA, 4416 bp, synthetic construct
  misc_feature 1..4416: note = FMC28z-SRG_FFF nucleic acid sequence
  source 1..4416: mol_type = other DNA
atgctgctgctggtcacatctctgctgctgtgcgagctgccccatcctgcctttctgctgatccccgacatccagatgacccagaccacaagcagcctgtctgccagcctgggcgatagagtgaccatcagctgtagagccagccaggacatcagcaagtacctgaactggtatcagcaaaagcccgacggcaccgtgaagctgctgatctaccacaccagcagactgcacagcggcgtgccaagcagattttctggcagcggctctggcaccgactacagcctgaccatctccaacctggaacaagaggacattgccacctacttttgccagcaaggcaacaccctgccttacacctttggcggaggcaccaagctggaaatcaccggctctacaagcggcagcggcaaacctggatctggcgagggatctaccaagggcgaagtgaaactgcaagagtctggccctggactggtggccccatctcagtctctgagcgtgacctgtacagtcagcggagtgtccctgcctgattacggcgtgtcctggatcagacagcctcctcggaaaggcctggaatggctgggagtgatctggggcagcgagacaacctactacaacagcgccctgaagtcccggctgaccatcatcaaggacaactccaagagccaggtgttcctgaagatgaacagcctgcagaccgacgacaccgccatctactattgcgccaagcactactactacggcggcagctacgctatggactattggggccagggcaccagcgtgacagtttcttctgccgccgctatcgaagtgatgtaccctccaccttacctggacaacgagaagtccaacggcaccatcatccatgtgaagggcaaacatctgtgcccctctccactgttccccggacctagcaagcctttctgggtgctcgttgttgttggcggcgtgctggcctgttatagcctgctggttaccgtggccttcatcatcttttgggtccgaagcaagagaagccggctgctgcacagcgactacatgaacatgacccctagacggcccggaccaaccagaaagcactaccagccttacgctcctcctagagacttcgccgcctaccggtccagagtgaagttcagcagatccgccgatgctcccgcctatcagcagggccagaaccagctgtacaacgagctgaacctggggagaagagaagagtacgacgtgctggacaagcggagaggacgcgatcctgaaatgggcggcaagcctcggagaaagaatccccaagagggactgtataatgagctgcagaaagacaagatggccgaggcctacagcgagatcggcatgaagggcgagcgcagaagaggcaaaggacacgatggcctgtatcagggcctgagcaccgccactaaggacacctacgatgcactgcacatgcaggccctgcctccaagaagggccaaaagaggatcaggcgaaggcagaggcagcctgctgacatgcggagatgtggaagagaaccccggaccagatcacctgggcgcttctctgtggcctcaagtgggatctctgtgtctgctgcttgctggcgctgcttgggctcctcctcctaatctgcccgatcctaagttcgagagcaaggccgctctgctggctgctagaggacctgaggaactgctgtgcttcaccgagagactcgaggacctcgtgtgcttctgggaagaagctgcttctgccggcgttggccctggcaattacagcttcagctaccagctggaagatgagccctggaagctgtgcagactgcatcaggcccctacagctagaggcgctgtgcggttttggtgtagcctgcctacagccgacaccagcagcttcgtgcctctggaactgagagtgacagccgcttctggcgcccctagataccacagagtgatccacatcaacgaggtggtgctgctggatgcccctgttggactggttgccagactggccgatgagtctggacatgtggtgctgagatggctgcctcctccagagacacctatgaccagccacatcagatacgaggtggacgtgtccgccggaaatggcgctggatctgtgcagagagtggaaatcctggaaggccggaccgagtgcgtgctgagcaatctgagaggcagaacccggtacaccttcgccgtcagagccagaatggctgagcctagctttggcggcttttggagcgcttggagcgagccagttagcctgctgacacctagcgatctggaccccgtggttatctctgttggctccatgggattgattatcagccttctctgtgtgtatttctggctggaacggacgatgccccgaattcccaccctgaagaacctagaggatcttgttactgaataccacgggaacttttcggcctggagtggtgtgtctaagggactggctgagagtctgcagccagactacagtgaacgactctgcctcgtcagtgagattcccccaaaaggaggggcccttggggaggggcctggggcctccccatgcaaccagcatagcccctactgggcccccccatgttacaccctaaagcctgaaaccagaagaaagcgcggaaagcctattccaaatccactcctcggcctggacagcacatctggatctggcgccaccaacttcagtctgctgaaacaggccggcgacgtcgaggaaaatcccgggccagatcatctcggagccagtctctggccacaagtcggaagcctgtgtttgttgctggctggtgcagcatgggccccaccaccaaatctccctgatccaaagtttgagtccaaagctgccctgctggccgcaagaggtcccgaagaactcctgtgttttacagagcggcttgaggatctcgtctgtttttgggaagaagccgcctccgctggcgtcggacccggcaattattcctttagctatcagctcgaggacgagccttggaaactgtgtcggctccaccaggctccaactgcaagaggcgccgttagattctggtgctctctgccaaccgccgataccagctcctttgtgcccctcgagcttagagtgactgctgctagcggagccccacggtatcatcgggtcatccatatcaatgaagtcgtcctgctggacgctcccgtgggacttgtcgctagactggctgacgaaagcggccacgttgtcctcagatggctcccacctcctgaaactcccatgacctctcacattcgctatgaagtggatgtctccgcaggcaacggtgccggaagcgttcagagagtcgagattctcgagggcagaacagagtgtgtgctgtctaacctgcggggcagaaccagatacacatttgctgtgcgcgccaggatggccgaaccttccttcggtggattttggagtgcttggagtgaacccgtgtctctgctgaccccttccgacctcgatcctattccgtggctcggccacctcctcgtgggcctcagcggggcttttggcttcatcatcttagtgtacttgctgatcaactgcaggaacaccgggccatggctgaagaaggtcctgaagtgtaacaccccagacccctcgaagttcttttcccagctgagctcagagcatggaggagacgtccagaagtggctctcttcgcccttcccctcatcgtccttcagccctggcggcctggcacctgagatctcgccactagaagtgctggagagggacaaggtgacgcagctgctcctgcagcaggacaaggtgcctgagcccgcatccttaagcagcaaccactcgctgaccagctgcttcaccaaccagggttacttcttcttccacctcccggatgccttggagatagaggcctgccaggtgttctttactttcgaccccttctcagaggaagaccctgatgagggtgtggccggggcacccacagggtcttccccccaacccctgcagcctctgtcaggggaggacgacgcctactgcaccttcccctccagggatgacctgctgctcttctcccccagtctcctcggtggccccagccccccaagcactgcccctgggggcagtggggccggtgaagagaggatgcccccttctttgcaagaaagagtccccagagactgggacccccagcccctggggcctcccaccccaggagtcccagacctggtggattttcagccaccccctgagctggtgctgcgagaggctggggaggaggtccctgacgctggccccagggagggagtcagtttcccctggtccaggcctcctgggcagggggagttcagggcccttaatgctcgcctgcccctgaacactgatgcctacttgtccctccaagaactccagggtcaggacccaactcacttggtgtag

SEQ ID NO: 61 - DNA, 43 bp, synthetic construct
  misc_feature 1..43: note = FMC63SRG-FMC_M5InfFwd primer
  source 1..43: mol_type = other DNA
gagctcggatctcacgtgccaccatgctgctgctggtcacatc

SEQ ID NO: 62 - DNA, 67 bp, synthetic construct
  misc_feature 1..67: note = FMC63SRG-FMC_M5InfRev primer
  source 1..67: mol_type = other DNA
tgtcagcaggctgcctctgccttcgcctgatcctcttttggcccttcttggaggcagggcctgcatg

SEQ ID NO: 63 - DNA, 66 bp, synthetic construct
  misc_feature 1..66: note = FMC63SRG-SRG_M5InfFwd primer
  source 1..66: mol_type = other DNA
ggcagcctgctgacatgcggagatgtggaagagaaccccggaccagatcacctgggcgcttctctg

SEQ ID NO: 64 - protein, 437 aa, synthetic construct
  REGION 1..437: note = EpoRm amino acid sequence
DHLGASLWPQVGSLCLLLAGAAWAPPPNLPDPKFESKAALLAARGPEELLCFTERLEDLVCFWEEAASAGVGPGNYSFSYQLEDEPWKLCRLHQAPTARGAVRFWCSLPTADTSSFVPLELRVTAASGAPRYHRVIHINEVVLLDAPVGLVARLADESGHVVLRWLPPPETPMTSHIRYEVDVSAGNGAGSVQRVEILEGRTECVLSNLRGRTRYTFAVRARMAEPSFGGFWSAWSEPVSLLTPSDLDPLILTLSLILVVILVLLTVLALLSHRRALKQKIWPGIPSPESEFEGLFTTHKGNFQLWLYQNDGCLWWSPCTPFTEDPPASLEVLSERCWGTMQAVEPGTDDEGPLLEPVGSEHAQDTYLVLDKWLLPRNPPSEDLPGPGGSVDIVAMDEGSEASSCSSALASKPSPEGASAASFEYTILDPSSQLLRP

SEQ ID NO: 65 - DNA, 1314 bp, synthetic construct
  misc_feature 1..1314: note = EpoRm nucleic acid sequence
  source 1..1314: mol_type = other DNA
gatcacctgggcgcttctctgtggcctcaagtgggatctctgtgtctgctgcttgctggcgctgcttgggctcctcctcctaatctgcccgatcctaagttcgagagcaaggccgctctgctggctgctagaggacctgaggaactgctgtgcttcaccgagcggctggaagatctcgtgtgcttctgggaagaagccgcctctgcaggcgttggccctggcaattacagcttcagctaccagcttgaggacgagccctggaagctgtgcagactgcatcaggcccctacagctagaggcgctgtgcggttttggtgtagcctgcctacagccgacaccagcagcttcgttcctctggaactgagagtgacagctgcctctggcgcccctagataccacagagtgatccacatcaacgaggtggtgctgctggatgcccctgttggactggttgccagactggccgatgagtctggacatgtggtgctgagatggctgcctcctccagagacacctatgaccagccacatcagatacgaggtggacgtgtccgccggaaatggcgctggatctgtgcagagagtggaaatcctggaaggccggaccgagtgcgtgctgagcaatctgagaggcagaacccggtacaccttcgccgtcagagccagaatggctgagcctagctttggcggcttttggagcgcttggagcgagccagttagcctgctgacacctagcgatctggaccctctgatcctgacactgagcctgatcctggtggtcatcctggtcctgctgactgttctggccctgctgtctcatcggagagccctgaagcagaagatctggcctggcatcccatctccagagagcgagttcgagggcctgttcaccacacacaagggcaacttccagctgtggctgtaccagaacgacggctgtctttggtggtccccttgcacacccttcacagaggaccctccagcctctctggaagtgctgagcgagagatgttggggcacaatgcaggccgtggaacccggcacagatgatgagggacctctgctggaacctgtgggatctgaacacgcccaggacacctacctggtgctggataagtggctgctgccccggaatcctccaagcgaagatttgcctggacctggcggctccgtggacatcgtggctatggatgaaggcagcgaggccagcagctgttcttctgccctggcctctaagccttctccagaaggcgcttctgccgccagcttcgagtacaccattctggacccaagctctcagctgctgaggccctaa

SEQ ID NO: 66 - protein, 708 aa, synthetic construct
  REGION 1..708: note = ZG-EpoRm amino acid sequence
MAQSKHGLTKEMTMKYRMEGCVDGHKFVITGEGIGYPFKGKQAINLCVVEGGPLPFAEDILSAAFMYGNRVFTEYPQDIVDYFKNSCPAGYTWDRSFLFEDGAVCICNADITVSVEENCMYHESKFYGVNFPADGPVMKKMTDNWEPSCEKIIPVPKQGILKGDVSMYLLLKDGGRLRCQFDTVYKAKSVPRKMPDWHFIQHKLTREDRSDAKNQKWHLTEHAIASGSALPRAKRGKPIPNPLLGLDSTSGSGEGRGSLLTCGDVEENPGPDHLGASLWPQVGSLCLLLAGAAWAPPPNLPDPKFESKAALLAARGPEELLCFTERLEDLVCFWEEAASAGVGPGNYSFSYQLEDEPWKLCRLHQAPTARGAVRFWCSLPTADTSSFVPLELRVTAASGAPRYHRVIHINEVVLLDAPVGLVARLADESGHVVLRWLPPPETPMTSHIRYEVDVSAGNGAGSVQRVEILEGRTECVLSNLRGRTRYTFAVRARMAEPSFGGFWSAWSEPVSLLTPSDLDPLILTLSLILVVILVLLTVLALLSHRRALKQKIWPGIPSPESEFEGLFTTHKGNFQLWLYQNDGCLWWSPCTPFTEDPPASLEVLSERCWGTMQAVEPGTDDEGPLLEPVGSEHAQDTYLVLDKWLLPRNPPSEDLPGPGGSVDIVAMDEGSEASSCSSALASKPSPEGASAASFEYTILDPSSQLLRP

SEQ ID NO: 67 - DNA, 2127 bp, synthetic construct
  misc_feature 1..2127: note = ZG-EpoRm nucleic acid sequence
  source 1..2127: mol_type = other DNA
atggcccagtccaagcacggcctgaccaaggagatgaccatgaagtaccgcatggagggctgcgtggacggccacaagttcgtgatcaccggcgagggcatcggctaccccttcaagggcaagcaggccatcaacctgtgcgtggtggagggcggccccttgcccttcgccgaggacatcttgtccgccgccttcatgtacggcaaccgcgtgttcaccgagtacccccaggacatcgtcgactacttcaagaactcctgccccgccggctacacctgggaccgctccttcctgttcgaggacggcgccgtgtgcatctgcaacgccgacatcaccgtgagcgtggaggagaactgcatgtaccacgagtccaagttctacggcgtgaacttccccgccgacggccccgtgatgaagaagatgaccgacaactgggagccctcctgcgagaagatcatccccgtgcccaagcagggcatcttgaagggcgacgtgagcatgtacctgctgctgaaggacggtggccgcttgcgctgccagttcgacaccgtgtacaaggccaagtccgtgccccgcaagatgcccgactggcacttcatccagcacaagctgacccgcgaggaccgcagcgacgccaagaaccagaagtggcacctgaccgagcacgccatcgcctccggctccgccttgcccagggccaagaggggcaagcccattcctaatcctctgctgggcctcgatagcacaagcggcagcggagaaggcagaggctctctgcttacatgcggcgacgtggaagagaaccccggacctgatcacctgggcgcttctctgtggcctcaagtgggatctctgtgtctgctgcttgctggcgctgcttgggctcctcctcctaatctgcccgatcctaagttcgagagcaaggccgctctgctggctgctagaggacctgaggaactgctgtgcttcaccgagcggctggaagatctcgtgtgcttctgggaagaagccgcctctgcaggcgttggccctggcaattacagcttcagctaccagcttgaggacgagccctggaagctgtgcagactgcatcaggcccctacagctagaggcgctgtgcggttttggtgtagcctgcctacagccgacaccagcagcttcgttcctctggaactgagagtgacagctgcctctggcgcccctagataccacagagtgatccacatcaacgaggtggtgctgctggatgcccctgttggactggttgccagactggccgatgagtctggacatgtggtgctgagatggctgcctcctccagagacacctatgaccagccacatcagatacgaggtggacgtgtccgccggaaatggcgctggatctgtgcagagagtggaaatcctggaaggccggaccgagtgcgtgctgagcaatctgagaggcagaacccggtacaccttcgccgtcagagccagaatggctgagcctagctttggcggcttttggagcgcttggagcgagccagttagcctgctgacacctagcgatctggaccctctgatcctgacactgagcctgatcctggtggtcatcctggtcctgctgactgttctggccctgctgtctcatcggagagccctgaagcagaagatctggcctggcatcccatctccagagagcgagttcgagggcctgttcaccacacacaagggcaacttccagctgtggctgtaccagaacgacggctgtctttggtggtccccttgcacacccttcacagaggaccctccagcctctctggaagtgctgagcgagagatgttggggcacaatgcaggccgtggaacccggcacagatgatgagggacctctgctggaacctgtgggatctgaacacgcccaggacacctacctggtgctggataagtggctgctgccccggaatcctccaagcgaagatttgcctggacctggcggctccgtggacatcgtggctatggatgaaggcagcgaggccagcagctgttcttctgccctggcctctaagccttctccagaaggcgcttctgccgccagcttcgagtacaccattctggacccaagctctcagctgctgaggccctaa

SEQ ID NO: 68 - DNA, 32 bp, synthetic construct
  misc_feature 1..32: note = ZGEpoRm-ZG_M5InfRev primer
  source 1..32: mol_type = other DNA
aggtccggggttctcttccacgtcgccgcatg

SEQ ID NO: 69 - DNA, 46 bp, synthetic construct
  misc_feature 1..46: note = ZGEpoRm-EpoRm_M5InfFwd primer
  source 1..46: mol_type = other DNA
gagaaccccggacctgatcacctgggcgcttctctgtggcctcaag

SEQ ID NO: 70 - DNA, 39 bp, synthetic construct
  misc_feature 1..39: note = ZGEpoRm-EpoRm_M5InfRev primer
  source 1..39: mol_type = other DNA
taacgtcgacggatccttagggcctcagcagctgagagc

SEQ ID NO: 71 - protein, 62 aa, Homo sapiens
KKVAKKPTNKAPHPKQEPQEINFPDDLPGSNTAAPVQETLHGCQPVTQEDGKESRISVQERQ

SEQ ID NO: 72 - DNA, 186 bp, Homo sapiens
  source 1..186: mol_type = genomic DNA
aaaaaggtggccaagaagccaaccaataaggccccccaccccaagcaggaaccccaggagatcaattttcccgacgatcttcctggctccaacactgctgctccagtgcaggagactttacatggatgccaaccggtcacccaggaggatggcaaagagagtcgcatctcagtgcaggagagacag

SEQ ID NO: 73 - protein, 551 aa, Homo sapiens
MAAPALSWRLPLLILLLPLATSWASAAVNGTSQFTCFYNSRANISCVWSQDGALQDTSCQVHAWPDRRRWNQTCELLPVSQASWACNLILGAPDSQKLTTVDIVTLRVLCREGVRWRVMAIQDFKPFENLRLMAPISLQVVHVETHRCNISWEISQASHYFERHLEFEARTLSPGHTWEEAPLLTLKQKQEWICLETLTPDTQYEFQVRVKPLQGEFTTWSPWSQPLAFRTKPAALGKDTIPWLGHLLVGLSGAFGFIILVYLLINCRNTGPWLKKVLKCNTPDPSKFFSQLSSEHGGDVQKWLSSPFPSSSFSPGGLAPEISPLEVLERDKVTQLLLQQDKVPEPASLSSNHSLTSCFTNQGYFFFHLPDALEIEACQVYFTYDPYSEEDPDEGVAGAPTGSSPQPLQPLSGEDDAYCTFPSRDDLLLFSPSLLGGPSPPSTAPGGSGAGEERMPPSLQERVPRDWDPQPLGPPTPGVPDLVDFQPPPELVLREAGEEVPDAGPREGVSFPWSRPPGQGEFRALNARLPLNTDAYLSLQELQGQDPTHLV

SEQ ID NO: 74 - protein, 369 aa, Homo sapiens
MLKPSLPFTSLLFLQLPLLGVGLNTTILTPNGNEDTTADFFLTTMPTDSLSVSTLPLPEVQCFVFNVEYMNCTWNSSSEPQPTNLTLHYWYKNSDNDKVQKCSHYLFSEEITSGCQLQKKEIHLYQTFVVQLQDPREPRRQATQMLKLQNLVIPWAPENLTLHKLSESQLELNWNNRFLNHCLEHLVQYRTDWDHSWTEQSVDYRHKFSLPSVDGQKRYTFRVRSRFNPLCGSAQHWSEWSHPIHWGSNTSKENPFLFALEAVVISVGSMGLIISLLCVYFWLERTMPRIPTLKNLEDLVTEYHGNFSAWSGVSKGLAESLQPDYSERLCLVSEIPPKGGALGEGPGASPCNQHSPYWAPPCYTLKPET